European Patent Specification EP 3 917 962 B1, published March 18, 2026. Title: Anti-IL2 Receptor Gamma Antigen-Binding Proteins. Applicant: Orengo, Jamie M Murphy, Andrew J. The sequence listing filed with the application follows.

SEQUENCE LISTING (386 sequences)

SEQ ID NO: 1 - DNA, 369 bp, Homo sapiens
caggtgcagctggtgcagtctggggctgaggtgaagaagcctggggcctcagtgcgggtctcctgcaaggcttctggatacaccttcaccgactacgatattcactgggtgcgacaggcccctggacatgggcttgagtggatggggtggatcaaccctaacagtggtggcacaaactatgcacagaagtttcagggcagggtcaccatgaccagggacacgtccatcagtacagtctacatggacctgagcaggctgagatctgacgacacggccgtgtattactgtgcgagagctgattatagtagttcgtattattattacggtatggacgtctggggccaagggaccacggtcaccgtctcctca

SEQ ID NO: 2 - protein, 123 aa, Homo sapiens
QVQLVQSGAEVKKPGASVRVSCKASGYTFTDYDIHWVRQAPGHGLEWMGWINPNSGGTNYAQKFQGRVTMTRDTSISTVYMDLSRLRSDDTAVYYCARADYSSSYYYYGMDVWGQGTTVTVSS

SEQ ID NO: 3 - DNA, 24 bp, Homo sapiens
ggatacaccttcaccgactacgat

SEQ ID NO: 4 - protein, 8 aa, Homo sapiens
GYTFTDYD

SEQ ID NO: 5 - DNA, 24 bp, Homo sapiens
atcaaccctaacagtggtggcaca

SEQ ID NO: 6 - protein, 8 aa, Homo sapiens
INPNSGGT

SEQ ID NO: 7 - DNA, 48 bp, Homo sapiens
gcgagagctgattatagtagttcgtattattattacggtatggacgtc

SEQ ID NO: 8 - protein, 16 aa, Homo sapiens
ARADYSSSYYYYGMDV

SEQ ID NO: 9 - DNA, 339 bp, Homo sapiens
gacatcgtgatgacccagtctccagactccctggctgtgtctctgggcgagagggccaccatcaactgcaagtccagccagagtgttttatacagctccaagaataagaactacttatcttggtaccagcagaaaccaggacagcctcctaagttgctcatttactgggcatctacccgggaattcggggtccctgaccgattcagtggccgcgggtctgggacagatttcactctcaccatcagcagcctgcaggctgaagatgtggcagtttattactgtcaacaatattatactactccgtacacttttggccaggggaccaagctggagatcaaa

SEQ ID NO: 10 - protein, 113 aa, Homo sapiens
DIVMTQSPDSLAVSLGERATINCKSSQSVLYSSKNKNYLSWYQQKPGQPPKLLIYWASTREFGVPDRFSGRGSGTDFTLTISSLQAEDVAVYYCQQYYTTPYTFGQGTKLEIK

SEQ ID NO: 11 - DNA, 36 bp, Homo sapiens
cagagtgttttatacagctccaagaataagaactac

SEQ ID NO: 12 - protein, 12 aa, Homo sapiens
QSVLYSSKNKNY

SEQ ID NO: 13 - DNA, 9 bp, Homo sapiens
tgggcatct

SEQ ID NO: 14 - protein, 3 aa, Homo sapiens
WAS

SEQ ID NO: 15 - DNA, 27 bp, Homo sapiens
caacaatattatactactccgtacact

SEQ ID NO: 16 - protein, 9 aa, Homo sapiens
QQYYTTPYT

SEQ ID NO: 17 - DNA, 1353 bp, Homo sapiens
caggtgcagctggtgcagtctggggctgaggtgaagaagcctggggcctcagtgcgggtctcctgcaaggcttctggatacaccttcaccgactacgatattcactgggtgcgacaggcccctggacatgggcttgagtggatggggtggatcaaccctaacagtggtggcacaaactatgcacagaagtttcagggcagggtcaccatgaccagggacacgtccatcagtacagtctacatggacctgagcaggctgagatctgacgacacggccgtgtattactgtgcgagagctgattatagtagttcgtattattattacggtatggacgtctggggccaagggaccacggtcaccgtctcctcagcctccaccaagggcccatcggtcttccccctggcgccctgctccaggagcacctccgagagcacagccgccctgggctgcctggtcaaggactacttccccgaaccggtgacggtgtcgtggaactcaggcgccctgaccagcggcgtgcacaccttcccggctgtcctacagtcctcaggactctactccctcagcagcgtggtgaccgtgccctccagcagcttgggcacgaagacctacacctgcaacgtagatcacaagcccagcaacaccaaggtggacaagagagttgagtccaaatatggtcccccatgcccaccctgcccagcacctgagttcctggggggaccatcagtcttcctgttccccccaaaacccaaggacactctcatgatctcccggacccctgaggtcacgtgcgtggtggtggacgtgagccaggaagaccccgaggtccagttcaactggtacgtggatggcgtggaggtgcataatgccaagacaaagccgcgggaggagcagttcaacagcacgtaccgtgtggtcagcgtcctcaccgtcctgcaccaggactggctgaacggcaaggagtacaagtgcaaggtctccaacaaaggcctcccgtcctccatcgagaaaaccatctccaaagccaaagggcagccccgagagccacaggtgtacaccctgcccccatcccaggaggagatgaccaagaaccaggtcagcctgacctgcctggtcaaaggcttctaccccagcgacatcgccgtggagtgggagagcaatgggcagccggagaacaactacaagaccacgcctcccgtgctggactccgacggctccttcttcctctacagcaggctcaccgtggacaagagcaggtggcaggaggggaatgtcttctcatgctccgtgatgcatgaggctctgcacaaccactacacacagaagtccctctccctgtctctgggtaaatga

SEQ ID NO: 18 - protein, 450 aa, Homo sapiens
QVQLVQSGAEVKKPGASVRVSCKASGYTFTDYDIHWVRQAPGHGLEWMGWINPNSGGTNYAQKFQGRVTMTRDTSISTVYMDLSRLRSDDTAVYYCARADYSSSYYYYGMDVWGQGTTVTVSSASTKGPSVFPLAPCSRSTSESTAALGCLVKDYFPEPVTVSWNSGALTSGVHTFPAVLQSSGLYSLSSVVTVPSSSLGTKTYTCNVDHKPSNTKVDKRVESKYGPPCPPCPAPEFLGGPSVFLFPPKPKDTLMISRTPEVTCVVVDVSQEDPEVQFNWYVDGVEVHNAKTKPREEQFNSTYRVVSVLTVLHQDWLNGKEYKCKVSNKGLPSSIEKTISKAKGQPREPQVYTLPPSQEEMTKNQVSLTCLVKGFYPSDIAVEWESNGQPENNYKTTPPVLDSDGSFFLYSRLTVDKSRWQEGNVFSCSVMHEALHNHYTQKSLSLSLGK

SEQ ID NO: 19 - DNA, 663 bp, Homo sapiens
gacatcgtgatgacccagtctccagactccctggctgtgtctctgggcgagagggccaccatcaactgcaagtccagccagagtgttttatacagctccaagaataagaactacttatcttggtaccagcagaaaccaggacagcctcctaagttgctcatttactgggcatctacccgggaattcggggtccctgaccgattcagtggccgcgggtctgggacagatttcactctcaccatcagcagcctgcaggctgaagatgtggcagtttattactgtcaacaatattatactactccgtacacttttggccaggggaccaagctggagatcaaacgaactgtggctgcaccatctgtcttcatcttcccgccatctgatgagcagttgaaatctggaactgcctctgttgtgtgcctgctgaataacttctatcccagagaggccaaagtacagtggaaggtggataacgccctccaatcgggtaactcccaggagagtgtcacagagcaggacagcaaggacagcacctacagcctcagcagcaccctgacgctgagcaaagcagactacgagaaacacaaagtctacgcctgcgaagtcacccatcagggcctgagctcgcccgtcacaaagagcttcaacaggggagagtgttag

SEQ ID NO: 20 - protein, 220 aa, Homo sapiens
DIVMTQSPDSLAVSLGERATINCKSSQSVLYSSKNKNYLSWYQQKPGQPPKLLIYWASTREFGVPDRFSGRGSGTDFTLTISSLQAEDVAVYYCQQYYTTPYTFGQGTKLEIKRTVAAPSVFIFPPSDEQLKSGTASVVCLLNNFYPREAKVQWKVDNALQSGNSQESVTEQDSKDSTYSLSSTLTLSKADYEKHKVYACEVTHQGLSSPVTKSFNRGEC

SEQ ID NO: 21 - DNA, 363 bp, Homo sapiens
caggtgcagctggtggagtctgggggaggcgtggtccagcctgggaggtccctgagactctcctgtacagcctctggattcaccttcagaagttatgacatgtactgggtccgccaggctccaggcaaggggctggagtgggtgtcagttataacatatgatggaaataataaatactatgcagactccgtgaagggccgattcaccatctccagagacaattccaagaacacgctatttctgcaaatgagcagcctgagacctgaggacacggctgtttattactgtgcgaaaaggggcttaatatgggtcggggagtcctttgactactggggccagggaaccctggtcaccgtctcctca

SEQ ID NO: 22 - protein, 121 aa, Homo sapiens
QVQLVESGGGVVQPGRSLRLSCTASGFTFRSYDMYWVRQAPGKGLEWVSVITYDGNNKYYADSVKGRFTISRDNSKNTLFLQMSSLRPEDTAVYYCAKRGLIWVGESFDYWGQGTLVTVSS

SEQ ID NO: 23 - DNA, 24 bp, Homo sapiens
ggattcaccttcagaagttatgac

SEQ ID NO: 24 - protein, 8 aa, Homo sapiens
GFTFRSYD

SEQ ID NO: 25 - DNA, 24 bp, Homo sapiens
ataacatatgatggaaataataaa

SEQ ID NO: 26 - protein, 8 aa, Homo sapiens
ITYDGNNK

SEQ ID NO: 27 - DNA, 42 bp, Homo sapiens
gcgaaaaggggcttaatatgggtcggggagtcctttgactac

SEQ ID NO: 28 - protein, 14 aa, Homo sapiens
AKRGLIWVGESFDY

SEQ ID NO: 29 - DNA, 321 bp, Homo sapiens
gacatccagatgacccagtctccttccaccctgtctgcatctgtaggagacagagtcaccatcacttgccgggccagtcagagtattaatagctggttggcctggtatcagcagaaaccagggaaagcccctaacctcctgatctataaggcgtctagtttagaaagtggggtcccatcaaggttcagcggcagtggatctgggacagaattcactctcaccatcagcagcctgcagcctgatgattttgcaacttattactgccaacagtataagagttattcgtggacgttcggccaagggaccaaggtggaaatcaaa

SEQ ID NO: 30 - protein, 107 aa, Homo sapiens
DIQMTQSPSTLSASVGDRVTITCRASQSINSWLAWYQQKPGKAPNLLIYKASSLESGVPSRFSGSGSGTEFTLTISSLQPDDFATYYCQQYKSYSWTFGQGTKVEIK

SEQ ID NO: 31 - DNA, 18 bp, Homo sapiens
cagagtattaatagctgg

SEQ ID NO: 32 - protein, 6 aa, Homo sapiens
QSINSW

SEQ ID NO: 33 - DNA, 9 bp, Homo sapiens
aaggcgtct

SEQ ID NO: 34 - protein, 3 aa, Homo sapiens
KAS

SEQ ID NO: 35 - DNA, 27 bp, Homo sapiens
caacagtataagagttattcgtggacg

SEQ ID NO: 36 - protein, 9 aa, Homo sapiens
QQYKSYSWT

SEQ ID NO: 37 - DNA, 1347 bp, Homo sapiens
caggtgcagctggtggagtctgggggaggcgtggtccagcctgggaggtccctgagactctcctgtacagcctctggattcaccttcagaagttatgacatgtactgggtccgccaggctccaggcaaggggctggagtgggtgtcagttataacatatgatggaaataataaatactatgcagactccgtgaagggccgattcaccatctccagagacaattccaagaacacgctatttctgcaaatgagcagcctgagacctgaggacacggctgtttattactgtgcgaaaaggggcttaatatgggtcggggagtcctttgactactggggccagggaaccctggtcaccgtctcctcagcctccaccaagggcccatcggtcttccccctggcgccctgctccaggagcacctccgagagcacagccgccctgggctgcctggtcaaggactacttccccgaaccggtgacggtgtcgtggaactcaggcgccctgaccagcggcgtgcacaccttcccggctgtcctacagtcctcaggactctactccctcagcagcgtggtgaccgtgccctccagcagcttgggcacgaagacctacacctgcaacgtagatcacaagcccagcaacaccaaggtggacaagagagttgagtccaaatatggtcccccatgcccaccctgcccagcacctgagttcctggggggaccatcagtcttcctgttccccccaaaacccaaggacactctcatgatctcccggacccctgaggtcacgtgcgtggtggtggacgtgagccaggaagaccccgaggtccagttcaactggtacgtggatggcgtggaggtgcataatgccaagacaaagccgcgggaggagcagttcaacagcacgtaccgtgtggtcagcgtcctcaccgtcctgcaccaggactggctgaacggcaaggagtacaagtgcaaggtctccaacaaaggcctcccgtcctccatcgagaaaaccatctccaaagccaaagggcagccccgagagccacaggtgtacaccctgcccccatcccaggaggagatgaccaagaaccaggtcagcctgacctgcctggtcaaaggcttctaccccagcgacatcgccgtggagtgggagagcaatgggcagccggagaacaactacaagaccacgcctcccgtgctggactccgacggctccttcttcctctacagcaggctcaccgtggacaagagcaggtggcaggaggggaatgtcttctcatgctccgtgatgcatgaggctctgcacaaccactacacacagaagtccctctccctgtctctgggtaaatga

SEQ ID NO: 38 - protein, 448 aa, Homo sapiens
QVQLVESGGGVVQPGRSLRLSCTASGFTFRSYDMYWVRQAPGKGLEWVSVITYDGNNKYYADSVKGRFTISRDNSKNTLFLQMSSLRPEDTAVYYCAKRGLIWVGESFDYWGQGTLVTVSSASTKGPSVFPLAPCSRSTSESTAALGCLVKDYFPEPVTVSWNSGALTSGVHTFPAVLQSSGLYSLSSVVTVPSSSLGTKTYTCNVDHKPSNTKVDKRVESKYGPPCPPCPAPEFLGGPSVFLFPPKPKDTLMISRTPEVTCVVVDVSQEDPEVQFNWYVDGVEVHNAKTKPREEQFNSTYRVVSVLTVLHQDWLNGKEYKCKVSNKGLPSSIEKTISKAKGQPREPQVYTLPPSQEEMTKNQVSLTCLVKGFYPSDIAVEWESNGQPENNYKTTPPVLDSDGSFFLYSRLTVDKSRWQEGNVFSCSVMHEALHNHYTQKSLSLSLGK

SEQ ID NO: 39 - DNA, 645 bp, Homo sapiens
gacatccagatgacccagtctccttccaccctgtctgcatctgtaggagacagagtcaccatcacttgccgggccagtcagagtattaatagctggttggcctggtatcagcagaaaccagggaaagcccctaacctcctgatctataaggcgtctagtttagaaagtggggtcccatcaaggttcagcggcagtggatctgggacagaattcactctcaccatcagcagcctgcagcctgatgattttgcaacttattactgccaacagtataagagttattcgtggacgttcggccaagggaccaaggtggaaatcaaacgaactgtggctgcaccatctgtcttcatcttcccgccatctgatgagcagttgaaatctggaactgcctctgttgtgtgcctgctgaataacttctatcccagagaggccaaagtacagtggaaggtggataacgccctccaatcgggtaactcccaggagagtgtcacagagcaggacagcaaggacagcacctacagcctcagcagcaccctgacgctgagcaaagcagactacgagaaacacaaagtctacgcctgcgaagtcacccatcagggcctgagctcgcccgtcacaaagagcttcaacaggggagagtgttag

SEQ ID NO: 40 - protein, 214 aa, Homo sapiens
DIQMTQSPSTLSASVGDRVTITCRASQSINSWLAWYQQKPGKAPNLLIYKASSLESGVPSRFSGSGSGTEFTLTISSLQPDDFATYYCQQYKSYSWTFGQGTKVEIKRTVAAPSVFIFPPSDEQLKSGTASVVCLLNNFYPREAKVQWKVDNALQSGNSQESVTEQDSKDSTYSLSSTLTLSKADYEKHKVYACEVTHQGLSSPVTKSFNRGEC

SEQ ID NO: 41 - DNA, 360 bp, Homo sapiens
caggtgcagctggtggagtctgggggaggcgtggtccagcctgggaggtccctgagactctcctgtgcagcctctggattcaacttcagaaactttggcatgcactgggtccgccaggctccaggcaaggggctggaatgggtggcaggtatattatatgatggaagtagtaaatactatgcagactccgtgaaggaccgattcaccatctccagagacaattccaagaacacgctgtttctgcaaatgaacagcctgagagctgaggacacggctatgtattactgtgcgaaagaggaggacacagccatggttccttttgattcctggggcccgggaaccctggtcaccgtctcctca

SEQ ID NO: 42 - protein, 120 aa, Homo sapiens
QVQLVESGGGVVQPGRSLRLSCAASGFNFRNFGMHWVRQAPGKGLEWVAGILYDGSSKYYADSVKDRFTISRDNSKNTLFLQMNSLRAEDTAMYYCAKEEDTAMVPFDSWGPGTLVTVSS

SEQ ID NO: 43 - DNA, 24 bp, Homo sapiens
ggattcaacttcagaaactttggc

SEQ ID NO: 44 - protein, 8 aa, Homo sapiens
GFNFRNFG

SEQ ID NO: 45 - DNA, 24 bp, Homo sapiens
atattatatgatggaagtagtaaa

SEQ ID NO: 46 - protein, 8 aa, Homo sapiens
ILYDGSSK

SEQ ID NO: 47 - DNA, 39 bp, Homo sapiens
gcgaaagaggaggacacagccatggttccttttgattcc

SEQ ID NO: 48 - protein, 13 aa, Homo sapiens
AKEEDTAMVPFDS

SEQ ID NO: 49 - DNA, 321 bp, Homo sapiens
gacatccagttgacccagtctccatccttcctgtctgcttctgtaggagacagagtcaccatcacttgctgggccagtcagggcattagtagttatttagcctggtatcagcaaaaaccagggaaagcccctaccctcctgatctatgctgcgtccactttgcaaagtggggtcccatcaaggttcagcggcagtggatctgggacagaattcactctcacaatcagcagcctgcagcctgaagattttgcaagttattactgtcaacagcttaagagttacccgctcactttcggcggagggaccaaggtggagatcaaa

SEQ ID NO: 50 - protein, 107 aa, Homo sapiens
DIQLTQSPSFLSASVGDRVTITCWASQGISSYLAWYQQKPGKAPTLLIYAASTLQSGVPSRFSGSGSGTEFTLTISSLQPEDFASYYCQQLKSYPLTFGGGTKVEIK

SEQ ID NO: 51 - DNA, 18 bp, Homo sapiens
cagggcattagtagttat

SEQ ID NO: 52 - protein, 6 aa, Homo sapiens
QGISSY

SEQ ID NO: 53 - DNA, 9 bp, Homo sapiens
gctgcgtcc

SEQ ID NO: 54 - protein, 3 aa, Homo sapiens
AAS

SEQ ID NO: 55 - DNA, 27 bp, Homo sapiens
caacagcttaagagttacccgctcact

SEQ ID NO: 56 - protein, 9 aa, Homo sapiens
QQLKSYPLT

SEQ ID NO: 57 - DNA, 1344 bp, Homo sapiens
caggtgcagctggtggagtctgggggaggcgtggtccagcctgggaggtccctgagactctcctgtgcagcctctggattcaacttcagaaactttggcatgcactgggtccgccaggctccaggcaaggggctggaatgggtggcaggtatattatatgatggaagtagtaaatactatgcagactccgtgaaggaccgattcaccatctccagagacaattccaagaacacgctgtttctgcaaatgaacagcctgagagctgaggacacggctatgtattactgtgcgaaagaggaggacacagccatggttccttttgattcctggggcccgggaaccctggtcaccgtctcctcagcctccaccaagggcccatcggtcttccccctggcgccctgctccaggagcacctccgagagcacagccgccctgggctgcctggtcaaggactacttccccgaaccggtgacggtgtcgtggaactcaggcgccctgaccagcggcgtgcacaccttcccggctgtcctacagtcctcaggactctactccctcagcagcgtggtgaccgtgccctccagcagcttgggcacgaagacctacacctgcaacgtagatcacaagcccagcaacaccaaggtggacaagagagttgagtccaaatatggtcccccatgcccaccctgcccagcacctgagttcctggggggaccatcagtcttcctgttccccccaaaacccaaggacactctcatgatctcccggacccctgaggtcacgtgcgtggtggtggacgtgagccaggaagaccccgaggtccagttcaactggtacgtggatggcgtggaggtgcataatgccaagacaaagccgcgggaggagcagttcaacagcacgtaccgtgtggtcagcgtcctcaccgtcctgcaccaggactggctgaacggcaaggagtacaagtgcaaggtctccaacaaaggcctcccgtcctccatcgagaaaaccatctccaaagccaaagggcagccccgagagccacaggtgtacaccctgcccccatcccaggaggagatgaccaagaaccaggtcagcctgacctgcctggtcaaaggcttctaccccagcgacatcgccgtggagtgggagagcaatgggcagccggagaacaactacaagaccacgcctcccgtgctggactccgacggctccttcttcctctacagcaggctcaccgtggacaagagcaggtggcaggaggggaatgtcttctcatgctccgtgatgcatgaggctctgcacaaccactacacacagaagtccctctccctgtctctgggtaaatga

SEQ ID NO: 58 - protein, 447 aa, Homo sapiens
QVQLVESGGGVVQPGRSLRLSCAASGFNFRNFGMHWVRQAPGKGLEWVAGILYDGSSKYYADSVKDRFTISRDNSKNTLFLQMNSLRAEDTAMYYCAKEEDTAMVPFDSWGPGTLVTVSSASTKGPSVFPLAPCSRSTSESTAALGCLVKDYFPEPVTVSWNSGALTSGVHTFPAVLQSSGLYSLSSVVTVPSSSLGTKTYTCNVDHKPSNTKVDKRVESKYGPPCPPCPAPEFLGGPSVFLFPPKPKDTLMISRTPEVTCVVVDVSQEDPEVQFNWYVDGVEVHNAKTKPREEQFNSTYRVVSVLTVLHQDWLNGKEYKCKVSNKGLPSSIEKTISKAKGQPREPQVYTLPPSQEEMTKNQVSLTCLVKGFYPSDIAVEWESNGQPENNYKTTPPVLDSDGSFFLYSRLTVDKSRWQEGNVFSCSVMHEALHNHYTQKSLSLSLGK

SEQ ID NO: 59 - DNA, 645 bp, Homo sapiens
gacatccagttgacccagtctccatccttcctgtctgcttctgtaggagacagagtcaccatcacttgctgggccagtcagggcattagtagttatttagcctggtatcagcaaaaaccagggaaagcccctaccctcctgatctatgctgcgtccactttgcaaagtggggtcccatcaaggttcagcggcagtggatctgggacagaattcactctcacaatcagcagcctgcagcctgaagattttgcaagttattactgtcaacagcttaagagttacccgctcactttcggcggagggaccaaggtggagatcaaacgaactgtggctgcaccatctgtcttcatcttcccgccatctgatgagcagttgaaatctggaactgcctctgttgtgtgcctgctgaataacttctatcccagagaggccaaagtacagtggaaggtggataacgccctccaatcgggtaactcccaggagagtgtcacagagcaggacagcaaggacagcacctacagcctcagcagcaccctgacgctgagcaaagcagactacgagaaacacaaagtctacgcctgcgaagtcacccatcagggcctgagctcgcccgtcacaaagagcttcaacaggggagagtgttag

SEQ ID NO: 60 - protein, 214 aa, Homo sapiens
DIQLTQSPSFLSASVGDRVTITCWASQGISSYLAWYQQKPGKAPTLLIYAASTLQSGVPSRFSGSGSGTEFTLTISSLQPEDFASYYCQQLKSYPLTFGGGTKVEIKRTVAAPSVFIFPPSDEQLKSGTASVVCLLNNFYPREAKVQWKVDNALQSGNSQESVTEQDSKDSTYSLSSTLTLSKADYEKHKVYACEVTHQGLSSPVTKSFNRGEC

SEQ ID NO: 61 - DNA, 366 bp, Homo sapiens
caggtgcagctgcaggagtcgggcccaggactggtgaagccttcacagaccctgtccctcacctgcactgtctctggtggctccatcagcagtggtggttactactggagctggatccgccagcacccagggaagggcctggagtggattggtttcatctattacagtgggaagacctactacaacccgtccctcaagagtcgacttaccatctcagtagacacgtctaagagccagttctccctgaagctgaggtctgtgactgccgcggacacggccgtgtattactgtgcgagactggggtataccaactcggccgggtggttcgacccctggggccagggaaccctggtcaccgtctcctca

SEQ ID NO: 62 - protein, 122 aa, Homo sapiens
QVQLQESGPGLVKPSQTLSLTCTVSGGSISSGGYYWSWIRQHPGKGLEWIGFIYYSGKTYYNPSLKSRLTISVDTSKSQFSLKLRSVTAADTAVYYCARLGYTNSAGWFDPWGQGTLVTVSS

SEQ ID NO: 63 - DNA, 30 bp, Homo sapiens
ggtggctccatcagcagtggtggttactac

SEQ ID NO: 64 - protein, 10 aa, Homo sapiens
GGSISSGGYY

SEQ ID NO: 65 - DNA, 21 bp, Homo sapiens
atctattacagtgggaagacc

SEQ ID NO: 66 - protein, 7 aa, Homo sapiens
IYYSGKT

SEQ ID NO: 67 - DNA, 42 bp, Homo sapiens
gcgagactggggtataccaactcggccgggtggttcgacccc

SEQ ID NO: 68 - protein, 14 aa, Homo sapiens
ARLGYTNSAGWFDP

SEQ ID NO: 69 - DNA, 321 bp, Homo sapiens
gacatccagatgacccagtctccatcctccctgtctgcatctgtaggagacagagtcaccatcacttgccgggcaagtcagagcattagcagctatttaaattggtatcagcagaaaccagggaaagcccctaacctcctgatctatgctgcatccagtttgcaaagtggggtcccatcaaggttcagtggcagtggatctgggacagatttcactctcaccatcagcagtctgcaacctgaagatcttgcaacttactactgtcaacagagttacacaaccccattcactttcggccctgggaccaaagtggatatcaaa

SEQ ID NO: 70 - protein, 107 aa, Homo sapiens
DIQMTQSPSSLSASVGDRVTITCRASQSISSYLNWYQQKPGKAPNLLIYAASSLQSGVPSRFSGSGSGTDFTLTISSLQPEDLATYYCQQSYTTPFTFGPGTKVDIK

SEQ ID NO: 71 - DNA, 18 bp, Homo sapiens
cagagcattagcagctat

SEQ ID NO: 72 - protein, 6 aa, Homo sapiens
QSISSY

SEQ ID NO: 73 - DNA, 9 bp, Homo sapiens
gctgcatcc

SEQ ID NO: 74 - DNA, 27 bp, Homo sapiens
caacagagttacacaaccccattcact

SEQ ID NO: 75 - protein, 9 aa, Homo sapiens
QQSYTTPFT

SEQ ID NO: 76 - DNA, 1350 bp, Homo sapiens
caggtgcagctgcaggagtcgggcccaggactggtgaagccttcacagaccctgtccctcacctgcactgtctctggtggctccatcagcagtggtggttactactggagctggatccgccagcacccagggaagggcctggagtggattggtttcatctattacagtgggaagacctactacaacccgtccctcaagagtcgacttaccatctcagtagacacgtctaagagccagttctccctgaagctgaggtctgtgactgccgcggacacggccgtgtattactgtgcgagactggggtataccaactcggccgggtggttcgacccctggggccagggaaccctggtcaccgtctcctcagcctccaccaagggcccatcggtcttccccctggcgccctgctccaggagcacctccgagagcacagccgccctgggctgcctggtcaaggactacttccccgaaccggtgacggtgtcgtggaactcaggcgccctgaccagcggcgtgcacaccttcccggctgtcctacagtcctcaggactctactccctcagcagcgtggtgaccgtgccctccagcagcttgggcacgaagacctacacctgcaacgtagatcacaagcccagcaacaccaaggtggacaagagagttgagtccaaatatggtcccccatgcccaccctgcccagcacctgagttcctggggggaccatcagtcttcctgttccccccaaaacccaaggacactctcatgatctcccggacccctgaggtcacgtgcgtggtggtggacgtgagccaggaagaccccgaggtccagttcaactggtacgtggatggcgtggaggtgcataatgccaagacaaagccgcgggaggagcagttcaacagcacgtaccgtgtggtcagcgtcctcaccgtcctgcaccaggactggctgaacggcaaggagtacaagtgcaaggtctccaacaaaggcctcccgtcctccatcgagaaaaccatctccaaagccaaagggcagccccgagagccacaggtgtacaccctgcccccatcccaggaggagatgaccaagaaccaggtcagcctgacctgcctggtcaaaggcttctaccccagcgacatcgccgtggagtgggagagcaatgggcagccggagaacaactacaagaccacgcctcccgtgctggactccgacggctccttcttcctctacagcaggctcaccgtggacaagagcaggtggcaggaggggaatgtcttctcatgctccgtgatgcatgaggctctgcacaaccactacacacagaagtccctctccctgtctctgggtaaatga

SEQ ID NO: 77 - protein, 449 aa, Homo sapiens
QVQLQESGPGLVKPSQTLSLTCTVSGGSISSGGYYWSWIRQHPGKGLEWIGFIYYSGKTYYNPSLKSRLTISVDTSKSQFSLKLRSVTAADTAVYYCARLGYTNSAGWFDPWGQGTLVTVSSASTKGPSVFPLAPCSRSTSESTAALGCLVKDYFPEPVTVSWNSGALTSGVHTFPAVLQSSGLYSLSSVVTVPSSSLGTKTYTCNVDHKPSNTKVDKRVESKYGPPCPPCPAPEFLGGPSVFLFPPKPKDTLMISRTPEVTCVVVDVSQEDPEVQFNWYVDGVEVHNAKTKPREEQFNSTYRVVSVLTVLHQDWLNGKEYKCKVSNKGLPSSIEKTISKAKGQPREPQVYTLPPSQEEMTKNQVSLTCLVKGFYPSDIAVEWESNGQPENNYKTTPPVLDSDGSFFLYSRLTVDKSRWQEGNVFSCSVMHEALHNHYTQKSLSLSLGK

SEQ ID NO: 78 - DNA, 645 bp, Homo sapiens
gacatccagatgacccagtctccatcctccctgtctgcatctgtaggagacagagtcaccatcacttgccgggcaagtcagagcattagcagctatttaaattggtatcagcagaaaccagggaaagcccctaacctcctgatctatgctgcatccagtttgcaaagtggggtcccatcaaggttcagtggcagtggatctgggacagatttcactctcaccatcagcagtctgcaacctgaagatcttgcaacttactactgtcaacagagttacacaaccccattcactttcggccctgggaccaaagtggatatcaaacgaactgtggctgcaccatctgtcttcatcttcccgccatctgatgagcagttgaaatctggaactgcctctgttgtgtgcctgctgaataacttctatcccagagaggccaaagtacagtggaaggtggataacgccctccaatcgggtaactcccaggagagtgtcacagagcaggacagcaaggacagcacctacagcctcagcagcaccctgacgctgagcaaagcagactacgagaaacacaaagtctacgcctgcgaagtcacccatcagggcctgagctcgcccgtcacaaagagcttcaacaggggagagtgttag

SEQ ID NO: 79 - protein, 214 aa, Homo sapiens
DIQMTQSPSSLSASVGDRVTITCRASQSISSYLNWYQQKPGKAPNLLIYAASSLQSGVPSRFSGSGSGTDFTLTISSLQPEDLATYYCQQSYTTPFTFGPGTKVDIKRTVAAPSVFIFPPSDEQLKSGTASVVCLLNNFYPREAKVQWKVDNALQSGNSQESVTEQDSKDSTYSLSSTLTLSKADYEKHKVYACEVTHQGLSSPVTKSFNRGEC

SEQ ID NO: 80 - DNA, 375 bp, Homo sapiens
gaggtgcagctggtggagtcggggggaggtttggtaaagcctggggggtcccttagactctcctgtgcagcctctggattcactttcagtaccgcctggatgagctgggtccgccagtctccagggagggggctggagtgggttggccgtatgaaaagcaagactgatggtgggacaacattctacgctgcacccgtgaaaggcagattcaccatctcaagagatgattcaaaaaacacactgtatctgcaaatgaacagcctgaaaaccgaggacacagccgtttattactgtaccacaggattagtcccggccttctataagtactacggcgtggacgtctggggccaagggaccacggtcaccgtctcctca

SEQ ID NO: 81 - protein, 125 aa, Homo sapiens
EVQLVESGGGLVKPGGSLRLSCAASGFTFSTAWMSWVRQSPGRGLEWVGRMKSKTDGGTTFYAAPVKGRFTISRDDSKNTLYLQMNSLKTEDTAVYYCTTGLVPAFYKYYGVDVWGQGTTVTVSS

SEQ ID NO: 82 - DNA, 24 bp, Homo sapiens
ggattcactttcagtaccgcctgg

SEQ ID NO: 83 - protein, 8 aa, Homo sapiens
GFTFSTAW

SEQ ID NO: 84 - DNA, 30 bp, Homo sapiens
atgaaaagcaagactgatggtgggacaaca

SEQ ID NO: 85 - protein, 10 aa, Homo sapiens
MKSKTDGGTT

SEQ ID NO: 86 - DNA, 48 bp, Homo sapiens
accacaggattagtcccggccttctataagtactacggcgtggacgtc

SEQ ID NO: 87 - protein, 16 aa, Homo sapiens
TTGLVPAFYKYYGVDV

SEQ ID NO: 88 - DNA, 318 bp, Homo sapiens
gacatccagatgacccagtctccatcctccctgtctgcatctgtaggagacagaatcaccatcacttgccaggcgagtcaggacattaccaactatttaaattggtatcagcagaagccagggaaagcccctaacctcctgatctacgatgcatccaatttggttacaggggtcccatcaaggttcagtggaagtggatctgggacagattttactttcaccatcctcagcctgcagcctgaagatattgcaacatattactgtcaacagtatgatagtctcctcactttcggccctgggaccaaagtggatatcaaa

SEQ ID NO: 89 - protein, 106 aa, Homo sapiens
DIQMTQSPSSLSASVGDRITITCQASQDITNYLNWYQQKPGKAPNLLIYDASNLVTGVPSRFSGSGSGTDFTFTILSLQPEDIATYYCQQYDSLLTFGPGTKVDIK

SEQ ID NO: 90 - DNA, 18 bp, Homo sapiens
caggacattaccaactat

SEQ ID NO: 91 - protein, 6 aa, Homo sapiens
QDITNY

SEQ ID NO: 92 - DNA, 9 bp, Homo sapiens
gatgcatcc

SEQ ID NO: 93 - protein, 3 aa, Homo sapiens
DAS

SEQ ID NO: 94 - DNA, 24 bp, Homo sapiens
caacagtatgatagtctcctcact

SEQ ID NO: 95 - protein, 8 aa, Homo sapiens
QQYDSLLT

SEQ ID NO: 96 - DNA, 1359 bp, Homo sapiens
gaggtgcagctggtggagtcggggggaggtttggtaaagcctggggggtcccttagactctcctgtgcagcctctggattcactttcagtaccgcctggatgagctgggtccgccagtctccagggagggggctggagtgggttggccgtatgaaaagcaagactgatggtgggacaacattctacgctgcacccgtgaaaggcagattcaccatctcaagagatgattcaaaaaacacactgtatctgcaaatgaacagcctgaaaaccgaggacacagccgtttattactgtaccacaggattagtcccggccttctataagtactacggcgtggacgtctggggccaagggaccacggtcaccgtctcctcagcctccaccaagggcccatcggtcttccccctggcgccctgctccaggagcacctccgagagcacagccgccctgggctgcctggtcaaggactacttccccgaaccggtgacggtgtcgtggaactcaggcgccctgaccagcggcgtgcacaccttcccggctgtcctacagtcctcaggactctactccctcagcagcgtggtgaccgtgccctccagcagcttgggcacgaagacctacacctgcaacgtagatcacaagcccagcaacaccaaggtggacaagagagttgagtccaaatatggtcccccatgcccaccctgcccagcacctgagttcctggggggaccatcagtcttcctgttccccccaaaacccaaggacactctcatgatctcccggacccctgaggtcacgtgcgtggtggtggacgtgagccaggaagaccccgaggtccagttcaactggtacgtggatggcgtggaggtgcataatgccaagacaaagccgcgggaggagcagttcaacagcacgtaccgtgtggtcagcgtcctcaccgtcctgcaccaggactggctgaacggcaaggagtacaagtgcaaggtctccaacaaaggcctcccgtcctccatcgagaaaaccatctccaaagccaaagggcagccccgagagccacaggtgtacaccctgcccccatcccaggaggagatgaccaagaaccaggtcagcctgacctgcctggtcaaaggcttctaccccagcgacatcgccgtggagtgggagagcaatgggcagccggagaacaactacaagaccacgcctcccgtgctggactccgacggctccttcttcctctacagcaggctcaccgtggacaagagcaggtggcaggaggggaatgtcttctcatgctccgtgatgcatgaggctctgcacaaccactacacacagaagtccctctccctgtctctgggtaaatga

SEQ ID NO: 97 - protein, 452 aa, Homo sapiens
EVQLVESGGGLVKPGGSLRLSCAASGFTFSTAWMSWVRQSPGRGLEWVGRMKSKTDGGTTFYAAPVKGRFTISRDDSKNTLYLQMNSLKTEDTAVYYCTTGLVPAFYKYYGVDVWGQGTTVTVSSASTKGPSVFPLAPCSRSTSESTAALGCLVKDYFPEPVTVSWNSGALTSGVHTFPAVLQSSGLYSLSSVVTVPSSSLGTKTYTCNVDHKPSNTKVDKRVESKYGPPCPPCPAPEFLGGPSVFLFPPKPKDTLMISRTPEVTCVVVDVSQEDPEVQFNWYVDGVEVHNAKTKPREEQFNSTYRVVSVLTVLHQDWLNGKEYKCKVSNKGLPSSIEKTISKAKGQPREPQVYTLPPSQEEMTKNQVSLTCLVKGFYPSDIAVEWESNGQPENNYKTTPPVLDSDGSFFLYSRLTVDKSRWQEGNVFSCSVMHEALHNHYTQKSLSLSLGK

SEQ ID NO: 98 - DNA, 642 bp, Homo sapiens
gacatccagatgacccagtctccatcctccctgtctgcatctgtaggagacagaatcaccatcacttgccaggcgagtcaggacattaccaactatttaaattggtatcagcagaagccagggaaagcccctaacctcctgatctacgatgcatccaatttggttacaggggtcccatcaaggttcagtggaagtggatctgggacagattttactttcaccatcctcagcctgcagcctgaagatattgcaacatattactgtcaacagtatgatagtctcctcactttcggccctgggaccaaagtggatatcaaacgaactgtggctgcaccatctgtcttcatcttcccgccatctgatgagcagttgaaatctggaactgcctctgttgtgtgcctgctgaataacttctatcccagagaggccaaagtacagtggaaggtggataacgccctccaatcgggtaactcccaggagagtgtcacagagcaggacagcaaggacagcacctacagcctcagcagcaccctgacgctgagcaaagcagactacgagaaacacaaagtctacgcctgcgaagtcacccatcagggcctgagctcgcccgtcacaaagagcttcaacaggggagagtgttag

SEQ ID NO: 99 - protein, 213 aa, Homo sapiens
DIQMTQSPSSLSASVGDRITITCQASQDITNYLNWYQQKPGKAPNLLIYDASNLVTGVPSRFSGSGSGTDFTFTILSLQPEDIATYYCQQYDSLLTFGPGTKVDIKRTVAAPSVFIFPPSDEQLKSGTASVVCLLNNFYPREAKVQWKVDNALQSGNSQESVTEQDSKDSTYSLSSTLTLSKADYEKHKVYACEVTHQGLSSPVTKSFNRGEC

SEQ ID NO: 100 - DNA, 369 bp, Homo sapiens
gaggtgcagctggtggagtctgggggaggcttggtccagcctggggggtccctgagactctcctgtgcagcctctggattcaccttcaataactatgcaatgcactgggtccgccaggctcccgggaagggactggaatatgtttcatctattagtagtagtgggggtagcacatattatgaagactctgtgaagggcagattcaccatctccagagacaattccaagaacacgctgtatcttcaaatgggcagcctgagagctgaggacatggctgtgtattactgtgcgagatcattctatggttcggggacttattatgatacttttgatatgtggggccaagggacaatggtcaccgtctcttca

SEQ ID NO: 101 - protein, 123 aa, Homo sapiens
EVQLVESGGGLVQPGGSLRLSCAASGFTFNNYAMHWVRQAPGKGLEYVSSISSSGGSTYYEDSVKGRFTISRDNSKNTLYLQMGSLRAEDMAVYYCARSFYGSGTYYDTFDMWGQGTMVTVSS

SEQ ID NO: 102 - DNA, 24 bp, Homo sapiens
ggattcaccttcaataactatgca

SEQ ID NO: 103 - protein, 8 aa, Homo sapiens
GFTFNNYA

SEQ ID NO: 104 - DNA, 24 bp, Homo sapiens
attagtagtagtgggggtagcaca

SEQ ID NO: 105 - protein, 8 aa, Homo sapiens
ISSSGGST

SEQ ID NO: 106 - DNA, 48 bp, Homo sapiens
gcgagatcattctatggttcggggacttattatgatacttttgatatg

SEQ ID NO: 107 - protein, 16 aa, Homo sapiens
ARSFYGSGTYYDTFDM

SEQ ID NO: 108 - DNA, 321 bp, Homo sapiens
gacatccagatgacccagtctccatcctccctgtctgcatctataggagacagagtcaccatcacttgccgggcaagtcagagcattagcaggtatttaaattggtatcagcagaaaccagggaaagcccctaagctcctgatctatgctgcatccagtttgcaaagtggggtcccatcaaggttcagtgccagtggatctgggacagatttcactctcaccatcagcagtctgcaacctgaagattttgcaacttactactgtcaacagagttacagtaccccgttcacttttggccaggggaccaagctggagatcaaa

SEQ ID NO: 109 - protein, 107 aa, Homo sapiens
DIQMTQSPSSLSASIGDRVTITCRASQSISRYLNWYQQKPGKAPKLLIYAASSLQSGVPSRFSASGSGTDFTLTISSLQPEDFATYYCQQSYSTPFTFGQGTKLEIK

SEQ ID NO: 110 - DNA, 18 bp, Homo sapiens
cagagcattagcaggtat

SEQ ID NO: 111 - protein, 6 aa, Homo sapiens
QSISRY

SEQ ID NO: 112 - DNA, 27 bp, Homo sapiens
caacagagttacagtaccccgttcact

SEQ ID NO: 113 - protein, 9 aa, Homo sapiens
QQSYSTPFT

SEQ ID NO: 114 - DNA, 1353 bp, Homo sapiens
gaggtgcagctggtggagtctgggggaggcttggtccagcctggggggtccctgagactctcctgtgcagcctctggattcaccttcaataactatgcaatgcactgggtccgccaggctcccgggaagggactggaatatgtttcatctattagtagtagtgggggtagcacatattatgaagactctgtgaagggcagattcaccatctccagagacaattccaagaacacgctgtatcttcaaatgggcagcctgagagctgaggacatggctgtgtattactgtgcgagatcattctatggttcggggacttattatgatacttttgatatgtggggccaagggacaatggtcaccgtctcttcagcctccaccaagggcccatcggtcttccccctggcgccctgctccaggagcacctccgagagcacagccgccctgggctgcctggtcaaggactacttccccgaaccggtgacggtgtcgtggaactcaggcgccctgaccagcggcgtgcacaccttcccggctgtcctacagtcctcaggactctactccctcagcagcgtggtgaccgtgccctccagcagcttgggcacgaagacctacacctgcaacgtagatcacaagcccagcaacaccaaggtggacaagagagttgagtccaaatatggtcccccatgcccaccctgcccagcacctgagttcctggggggaccatcagtcttcctgttccccccaaaacccaaggacactctcatgatctcccggacccctgaggtcacgtgcgtggtggtggacgtgagccaggaagaccccgaggtccagttcaactggtacgtggatggcgtggaggtgcataatgccaagacaaagccgcgggaggagcagttcaacagcacgtaccgtgtggtcagcgtcctcaccgtcctgcaccaggactggctgaacggcaaggagtacaagtgcaaggtctccaacaaaggcctcccgtcctccatcgagaaaaccatctccaaagccaaagggcagccccgagagccacaggtgtacaccctgcccccatcccaggaggagatgaccaagaaccaggtcagcctgacctgcctggtcaaaggcttctaccccagcgacatcgccgtggagtgggagagcaatgggcagccggagaacaactacaagaccacgcctcccgtgctggactccgacggctccttcttcctctacagcaggctcaccgtggacaagagcaggtggcaggaggggaatgtcttctcatgctccgtgatgcatgaggctctgcacaaccactacacacagaagtccctctccctgtctctgggtaaatga

SEQ ID NO: 115 - protein, 450 aa, Homo sapiens
EVQLVESGGGLVQPGGSLRLSCAASGFTFNNYAMHWVRQAPGKGLEYVSSISSSGGSTYYEDSVKGRFTISRDNSKNTLYLQMGSLRAEDMAVYYCARSFYGSGTYYDTFDMWGQGTMVTVSSASTKGPSVFPLAPCSRSTSESTAALGCLVKDYFPEPVTVSWNSGALTSGVHTFPAVLQSSGLYSLSSVVTVPSSSLGTKTYTCNVDHKPSNTKVDKRVESKYGPPCPPCPAPEFLGGPSVFLFPPKPKDTLMISRTPEVTCVVVDVSQEDPEVQFNWYVDGVEVHNAKTKPREEQFNSTYRVVSVLTVLHQDWLNGKEYKCKVSNKGLPSSIEKTISKAKGQPREPQVYTLPPSQEEMTKNQVSLTCLVKGFYPSDIAVEWESNGQPENNYKTTPPVLDSDGSFFLYSRLTVDKSRWQEGNVFSCSVMHEALHNHYTQKSLSLSLGK

SEQ ID NO: 116 - DNA, 645 bp, Homo sapiens
gacatccagatgacccagtctccatcctccctgtctgcatctataggagacagagtcaccatcacttgccgggcaagtcagagcattagcaggtatttaaattggtatcagcagaaaccagggaaagcccctaagctcctgatctatgctgcatccagtttgcaaagtggggtcccatcaaggttcagtgccagtggatctgggacagatttcactctcaccatcagcagtctgcaacctgaagattttgcaacttactactgtcaacagagttacagtaccccgttcacttttggccaggggaccaagctggagatcaaacgaactgtggctgcaccatctgtcttcatcttcccgccatctgatgagcagttgaaatctggaactgcctctgttgtgtgcctgctgaataacttctatcccagagaggccaaagtacagtggaaggtggataacgccctccaatcgggtaactcccaggagagtgtcacagagcaggacagcaaggacagcacctacagcctcagcagcaccctgacgctgagcaaagcagactacgagaaacacaaagtctacgcctgcgaagtcacccatcagggcctgagctcgcccgtcacaaagagcttcaacaggggagagtgttag

SEQ ID NO: 117 - protein, 214 aa, Homo sapiens
DIQMTQSPSSLSASIGDRVTITCRASQSISRYLNWYQQKPGKAPKLLIYAASSLQSGVPSRFSASGSGTDFTLTISSLQPEDFATYYCQQSYSTPFTFGQGTKLEIKRTVAAPSVFIFPPSDEQLKSGTASVVCLLNNFYPREAKVQWKVDNALQSGNSQESVTEQDSKDSTYSLSSTLTLSKADYEKHKVYACEVTHQGLSSPVTKSFNRGEC

SEQ ID NO: 118 - DNA, 342 bp, Homo sapiens
caggtgcagctggtggagtctgggggagacttggtcaagcctggggggtccctgagactctcctgtgcaacctctggattcaccttcagtgacttttacatgacctggatccgccaggctccagggaagggattggagtggatttcatatataagtaatagtgggagtatcgtgaagtacgcagactctgtgaagggccgattcaccatttccagggataacgccaagaactcactgtatctgcaaatgaacagcctgagagccgaggacacggccatttattactgtgcgcggttttatggtgacagatggggccagggaaccctggtcaccgtctcctca

SEQ ID NO: 119 - protein, 114 aa, Homo sapiens
QVQLVESGGDLVKPGGSLRLSCATSGFTFSDFYMTWIRQAPGKGLEWISYISNSGSIVKYADSVKGRFTISRDNAKNSLYLQMNSLRAEDTAIYYCARFYGDRWGQGTLVTVSS

SEQ ID NO: 120 - DNA, 24 bp, Homo sapiens
ggattcaccttcagtgacttttac

SEQ ID NO: 121 - protein, 8 aa, Homo sapiens
GFTFSDFY

SEQ ID NO: 122 - DNA, 24 bp, Homo sapiens
ataagtaatagtgggagtatcgtg

SEQ ID NO: 123 - protein, 8 aa, Homo sapiens
ISNSGSIV

SEQ ID NO: 124 - DNA, 21 bp, Homo sapiens
gcgcggttttatggtgacaga

SEQ ID NO: 125 - protein, 7 aa, Homo sapiens
ARFYGDR

SEQ ID NO: 126 - DNA, 321 bp, Homo sapiens
gacatccagttgacccagtctccatctttcctgtctgcatctgtaggagacagagtcaccatcacttgctgggccagtcagggcattagcacttttttagcctggtatcagcaaaagccgggtaaagcccctaagctcctgatctatgctgcatctactttacaaagtggggtcccatcgcgattcagcggcagcggatctgggacagatttcactctcacaatcagcagcctgcagcctgaagattttgcaacttatcactgtcaacaacttaataattacccgtggacgttcggccaagggaccaaggtggaaatcaaa

SEQ ID NO: 127 - protein, 107 aa, Homo sapiens
DIQLTQSPSFLSASVGDRVTITCWASQGISTFLAWYQQKPGKAPKLLIYAASTLQSGVPSRFSGSGSGTDFTLTISSLQPEDFATYHCQQLNNYPWTFGQGTKVEIK

SEQ ID NO: 128 - DNA, 18 bp, Homo sapiens
cagggcattagcactttt

SEQ ID NO: 129 - protein, 6 aa, Homo sapiens
QGISTF

SEQ ID NO: 130 - DNA, 9 bp, Homo sapiens
gctgcatct

SEQ ID NO: 131 - DNA, 27 bp, Homo sapiens
caacaacttaataattacccgtggacg

SEQ ID NO: 132 - protein, 9 aa, Homo sapiens
QQLNNYPWT

SEQ ID NO: 133 - DNA, 1326 bp, Homo sapiens
caggtgcagctggtggagtctgggggagacttggtcaagcctggggggtccctgagactctcctgtgcaacctctggattcaccttcagtgacttttacatgacctggatccgccaggctccagggaagggattggagtggatttcatatataagtaatagtgggagtatcgtgaagtacgcagactctgtgaagggccgattcaccatttccagggataacgccaagaactcactgtatctgcaaatgaacagcctgagagccgaggacacggccatttattactgtgcgcggttttatggtgacagatggggccagggaaccctggtcaccgtctcctcagcctccaccaagggcccatcggtcttccccctggcgccctgctccaggagcacctccgagagcacagccgccctgggctgcctggtcaaggactacttccccgaaccggtgacggtgtcgtggaactcaggcgccctgaccagcggcgtgcacaccttcccggctgtcctacagtcctcaggactctactccctcagcagcgtggtgaccgtgccctccagcagcttgggcacgaagacctacacctgcaacgtagatcacaagcccagcaacaccaaggtggacaagagagttgagtccaaatatggtcccccatgcccaccctgcccagcacctgagttcctggggggaccatcagtcttcctgttccccccaaaacccaaggacactctcatgatctcccggacccctgaggtcacgtgcgtggtggtggacgtgagccaggaagaccccgaggtccagttcaactggtacgtggatggcgtggaggtgcataatgccaagacaaagccgcgggaggagcagttcaacagcacgtaccgtgtggtcagcgtcctcaccgtcctgcaccaggactggctgaacggcaaggagtacaagtgcaaggtctccaacaaaggcctcccgtcctccatcgagaaaaccatctccaaagccaaagggcagccccgagagccacaggtgtacaccctgcccccatcccaggaggagatgaccaagaaccaggtcagcctgacctgcctggtcaaaggcttctaccccagcgacatcgccgtggagtgggagagcaatgggcagccggagaacaactacaagaccacgcctcccgtgctggactccgacggctccttcttcctctacagcaggctcaccgtggacaagagcaggtggcaggaggggaatgtcttctcatgctccgtgatgcatgaggctctgcacaaccactacacacagaagtccctctccctgtctctgggtaaatga

SEQ ID NO: 134 - protein, 441 aa, Homo sapiens
QVQLVESGGDLVKPGGSLRLSCATSGFTFSDFYMTWIRQAPGKGLEWISYISNSGSIVKYADSVKGRFTISRDNAKNSLYLQMNSLRAEDTAIYYCARFYGDRWGQGTLVTVSSASTKGPSVFPLAPCSRSTSESTAALGCLVKDYFPEPVTVSWNSGALTSGVHTFPAVLQSSGLYSLSSVVTVPSSSLGTKTYTCNVDHKPSNTKVDKRVESKYGPPCPPCPAPEFLGGPSVFLFPPKPKDTLMISRTPEVTCVVVDVSQEDPEVQFNWYVDGVEVHNAKTKPREEQFNSTYRVVSVLTVLHQDWLNGKEYKCKVSNKGLPSSIEKTISKAKGQPREPQVYTLPPSQEEMTKNQVSLTCLVKGFYPSDIAVEWESNGQPENNYKTTPPVLDSDGSFFLYSRLTVDKSRWQEGNVFSCSVMHEALHNHYTQKSLSLSLGK

SEQ ID NO: 135 - DNA, 645 bp, Homo sapiens
gacatccagttgacccagtctccatctttcctgtctgcatctgtaggagacagagtcaccatcacttgctgggccagtcagggcattagcacttttttagcctggtatcagcaaaagccgggtaaagcccctaagctcctgatctatgctgcatctactttacaaagtggggtcccatcgcgattcagcggcagcggatctgggacagatttcactctcacaatcagcagcctgcagcctgaagattttgcaacttatcactgtcaacaacttaataattacccgtggacgttcggccaagggaccaaggtggaaatcaaacgaactgtggctgcaccatctgtcttcatcttcccgccatctgatgagcagttgaaatctggaactgcctctgttgtgtgcctgctgaataacttctatcccagagaggccaaagtacagtggaaggtggataacgccctccaatcgggtaactcccaggagagtgtcacagagcaggacagcaaggacagcacctacagcctcagcagcaccctgacgctgagcaaagcagactacgagaaacacaaagtctacgcctgcgaagtcacccatcagggcctgagctcgcccgtcacaaagagcttcaacaggggagagtgttag

SEQ ID NO: 136 - protein, 214 aa, Homo sapiens
DIQLTQSPSFLSASVGDRVTITCWASQGISTFLAWYQQKPGKAPKLLIYAASTLQSGVPSRFSGSGSGTDFTLTISSLQPEDFATYHCQQLNNYPWTFGQGTKVEIKRTVAAPSVFIFPPSDEQLKSGTASVVCLLNNFYPREAKVQWKVDNALQSGNSQESVTEQDSKDSTYSLSSTLTLSKADYEKHKVYACEVTHQGLSSPVTKSFNRGEC

SEQ ID NO: 137 - DNA, 342 bp, Homo sapiens
caggtgcagctggtggagtctgggggaggcttggtcaagcctggagggtccctgagactctcctgtgaagcctctggattcaccttcaatgacttctatatgacctggatccgccaggctccagggaaggggctggagtggattgcatacatttctaagagtggtgataaaatgcgttatgcagactctgtgaagggccgattcagcacctccagggacaacgccaagaattcactatccttgcaaatgaatagcctgagagccgaggacacggccgtgtattattgtgcgagattctacggtgatatatggggccagggaaccctggtcaccgtctcctca

SEQ ID NO: 138 - protein, 114 aa, Homo sapiens
QVQLVESGGGLVKPGGSLRLSCEASGFTFNDFYMTWIRQAPGKGLEWIAYISKSGDKMRYADSVKGRFSTSRDNAKNSLSLQMNSLRAEDTAVYYCARFYGDIWGQGTLVTVSS

SEQ ID NO: 139 - DNA, 24 bp, Homo sapiens
ggattcaccttcaatgacttctat

SEQ ID NO: 140 - protein, 8 aa, Homo sapiens
GFTFNDFY

SEQ ID NO: 141 - DNA, 24 bp, Homo sapiens
atttctaagagtggtgataaaatg

SEQ ID NO: 142 - protein, 8 aa, Homo sapiens
ISKSGDKM

SEQ ID NO: 143 - DNA, 21 bp, Homo sapiens
gcgagattctacggtgatata

SEQ ID NO: 144 - protein, 7 aa, Homo sapiens
ARFYGDI

SEQ ID NO: 145 - DNA, 321 bp, Homo sapiens
gacatccagttgacccagtctccatccttcctgtctgcatctgtaggagacagagtcaccatcacttgctgggccagtcaggacattagcagttttttagtctggtatcagcaaaaaccagggaaagcccctaacctcctgatctatgctgcatccgctttgcagagtggggtcccatcaaggttcagcggcagtggatctgggacagaattcactctcacaatcagcagcctgcagcctgaagattttgcaagttattactgtgaacagcttaataattatccgtggacgttcggccaagggaccaaggtggaaatcaaa

SEQ ID NO: 146 - protein, 107 aa, Homo sapiens
DIQLTQSPSFLSASVGDRVTITCWASQDISSFLVWYQQKPGKAPNLLIYAASALQSGVPSRFSGSGSGTEFTLTISSLQPEDFASYYCEQLNNYPWTFGQGTKVEIK

SEQ ID NO: 147 - DNA, 18 bp, Homo sapiens
caggacattagcagtttt

SEQ ID NO: 148 - protein, 6 aa, Homo sapiens
QDISSF

SEQ ID NO: 149 - DNA, 27 bp, Homo sapiens
gaacagcttaataattatccgtggacg

SEQ ID NO: 150 - protein, 9 aa, Homo sapiens
EQLNNYPWT

SEQ ID NO: 151 - DNA, 1326 bp, Homo sapiens
caggtgcagctggtggagtctgggggaggcttggtcaagcctggagggtccctgagactctcctgtgaagcctctggattcaccttcaatgacttctatatgacctggatccgccaggctccagggaaggggctggagtggattgcatacatttctaagagtggtgataaaatgcgttatgcagactctgtgaagggccgattcagcacctccagggacaacgccaagaattcactatccttgcaaatgaatagcctgagagccgaggacacggccgtgtattattgtgcgagattctacggtgatatatggggccagggaaccctggtcaccgtctcctcagcctccaccaagggcccatcggtcttccccctggcgccctgctccaggagcacctccgagagcacagccgccctgggctgcctggtcaaggactacttccccgaaccggtgacggtgtcgtggaactcaggcgccctgaccagcggcgtgcacaccttcccggctgtcctacagtcctcaggactctactccctcagcagcgtggtgaccgtgccctccagcagcttgggcacgaagacctacacctgcaacgtagatcacaagcccagcaacaccaaggtggacaagagagttgagtccaaatatggtcccccatgcccaccctgcccagcacctgagttcctggggggaccatcagtcttcctgttccccccaaaacccaaggacactctcatgatctcccggacccctgaggtcacgtgcgtggtggtggacgtgagccaggaagaccccgaggtccagttcaactggtacgtggatggcgtggaggtgcataatgccaagacaaagccgcgggaggagcagttcaacagcacgtaccgtgtggtcagcgtcctcaccgtcctgcaccaggactggctgaacggcaaggagtacaagtgcaaggtctccaacaaaggcctcccgtcctccatcgagaaaaccatctccaaagccaaagggcagccccgagagccacaggtgtacaccctgcccccatcccaggaggagatgaccaagaaccaggtcagcctgacctgcctggtcaaaggcttctaccccagcgacatcgccgtggagtgggagagcaatgggcagccggagaacaactacaagaccacgcctcccgtgctggactccgacggctccttcttcctctacagcaggctcaccgtggacaagagcaggtggcaggaggggaatgtcttctcatgctccgtgatgcatgaggctctgcacaaccactacacacagaagtccctctccctgtctctgggtaaatga

SEQ ID NO: 152 - protein, 441 aa, Homo sapiens
QVQLVESGGGLVKPGGSLRLSCEASGFTFNDFYMTWIRQAPGKGLEWIAYISKSGDKMRYADSVKGRFSTSRDNAKNSLSLQMNSLRAEDTAVYYCARFYGDIWGQGTLVTVSSASTKGPSVFPLAPCSRSTSESTAALGCLVKDYFPEPVTVSWNSGALTSGVHTFPAVLQSSGLYSLSSVVTVPSSSLGTKTYTCNVDHKPSNTKVDKRVESKYGPPCPPCPAPEFLGGPSVFLFPPKPKDTLMISRTPEVTCVVVDVSQEDPEVQFNWYVDGVEVHNAKTKPREEQFNSTYRVVSVLTVLHQDWLNGKEYKCKVSNKGLPSSIEKTISKAKGQPREPQVYTLPPSQEEMTKNQVSLTCLVKGFYPSDIAVEWESNGQPENNYKTTPPVLDSDGSFFLYSRLTVDKSRWQEGNVFSCSVMHEALHNHYTQKSLSLSLGK

SEQ ID NO: 153 - DNA, 645 bp, Homo sapiens
gacatccagttgacccagtctccatccttcctgtctgcatctgtaggagacagagtcaccatcacttgctgggccagtcaggacattagcagttttttagtctggtatcagcaaaaaccagggaaagcccctaacctcctgatctatgctgcatccgctttgcagagtggggtcccatcaaggttcagcggcagtggatctgggacagaattcactctcacaatcagcagcctgcagcctgaagattttgcaagttattactgtgaacagcttaataattatccgtggacgttcggccaagggaccaaggtggaaatcaaacgaactgtggctgcaccatctgtcttcatcttcccgccatctgatgagcagttgaaatctggaactgcctctgttgtgtgcctgctgaataacttctatcccagagaggccaaagtacagtggaaggtggataacgccctccaatcgggtaactcccaggagagtgtcacagagcaggacagcaaggacagcacctacagcctcagcagcaccctgacgctgagcaaagcagactacgagaaacacaaagtctacgcctgcgaagtcacccatcagggcctgagctcgcccgtcacaaagagcttcaacaggggagagtgttag

SEQ ID NO: 154 - protein, 214 aa, Homo sapiens
DIQLTQSPSFLSASVGDRVTITCWASQDISSFLVWYQQKPGKAPNLLIYAASALQSGVPSRFSGSGSGTEFTLTISSLQPEDFASYYCEQLNNYPWTFGQGTKVEIKRTVAAPSVFIFPPSDEQLKSGTASVVCLLNNFYPREAKVQWKVDNALQSGNSQESVTEQDSKDSTYSLSSTLTLSKADYEKHKVYACEVTHQGLSSPVTKSFNRGEC

SEQ ID NO: 155 - DNA, 375 bp, Homo sapiens
gaggtgcagctggtggagtccgggggacgcttggtacagcctggggggtccctgagactctcctgtgaagcctctggattcacgtttagtaattatggcatgacctgggtccgccaggctccagggaaggggctggaatgggtctcagttattagtggcagtgataatagaaaatactatgcagagtccgtgaagggccggttcaccatctccagagacaattccaaaaacacactatatctgcaaatgaatagcctgagagccgaggacacggccgtctattactgtgcaaaattgggatatagtcgttcgtccaaggacttctactacggaatggacgtctggggccaagggaccacggtcaccgtctcctca

SEQ ID NO: 156 - protein, 125 aa, Homo sapiens
EVQLVESGGRLVQPGGSLRLSCEASGFTFSNYGMTWVRQAPGKGLEWVSVISGSDNRKYYAESVKGRFTISRDNSKNTLYLQMNSLRAEDTAVYYCAKLGYSRSSKDFYYGMDVWGQGTTVTVSS

SEQ ID NO: 157 - DNA, 24 bp, Homo sapiens
ggattcacgtttagtaattatggc

SEQ ID NO: 158 - protein, 8 aa, Homo sapiens
GFTFSNYG

SEQ ID NO: 159 - DNA, 24 bp, Homo sapiens
attagtggcagtgataatagaaaa

SEQ ID NO: 160 - protein, 8 aa, Homo sapiens
ISGSDNRK

SEQ ID NO: 161 - DNA, 54 bp, Homo sapiens
gcaaaattgggatatagtcgttcgtccaaggacttctactacggaatggacgtc

SEQ ID NO: 162 - protein, 18 aa, Homo sapiens
AKLGYSRSSKDFYYGMDV

SEQ ID NO: 163 - DNA, 339 bp, Homo sapiens
gacatcgtgatgacccagtctccagactccctggctgtgtctctgggcgagagggccaccatcaactgcaagtccagccagagtgttttatacaattccaataataggaactacttagtttggtaccagcagaaaccaggacagtctcctaagttgctcatttactgggcatctacccgggaatccggggtccctgaccggttcagtggcagcgggtctgggacagatttcactctcaccatcagcagcctgcaggctgaagatgtggcagtgtattactgtcagcaatattataatgttccgtacacttttggccaggggaccaagctggagatcaaa

SEQ ID NO: 164 - protein, 113 aa, Homo sapiens
DIVMTQSPDSLAVSLGERATINCKSSQSVLYNSNNRNYLVWYQQKPGQSPKLLIYWASTRESGVPDRFSGSGSGTDFTLTISSLQAEDVAVYYCQQYYNVPYTFGQGTKLEIK

SEQ ID NO: 165 - DNA, 36 bp, Homo sapiens
cagagtgttttatacaattccaataataggaactac

SEQ ID NO: 166 - protein, 12 aa, Homo sapiens
QSVLYNSNNRNY

SEQ ID NO: 167 - DNA, 27 bp, Homo sapiens
cagcaatattataatgttccgtacact

SEQ ID NO: 168 - protein, 9 aa, Homo sapiens
QQYYNVPYT

SEQ ID NO: 169 - DNA, 1359 bp, Homo sapiens
gaggtgcagctggtggagtccgggggacgcttggtacagcctggggggtccctgagactctcctgtgaagcctctggattcacgtttagtaattatggcatgacctgggtccgccaggctccagggaaggggctggaatgggtctcagttattagtggcagtgataatagaaaatactatgcagagtccgtgaagggccggttcaccatctccagagacaattccaaaaacacactatatctgcaaatgaatagcctgagagccgaggacacggccgtctattactgtgcaaaattgggatatagtcgttcgtccaaggacttctactacggaatggacgtctggggccaagggaccacggtcaccgtctcctcagcctccaccaagggcccatcggtcttccccctggcgccctgctccaggagcacctccgagagcacagccgccctgggctgcctggtcaaggactacttccccgaaccggtgacggtgtcgtggaactcaggcgccctgaccagcggcgtgcacaccttcccggctgtcctacagtcctcaggactctactccctcagcagcgtggtgaccgtgccctccagcagcttgggcacgaagacctacacctgcaacgtagatcacaagcccagcaacaccaaggtggacaagagagttgagtccaaatatggtcccccatgcccaccctgcccagcacctgagttcctggggggaccatcagtcttcctgttccccccaaaacccaaggacactctcatgatctcccggacccctgaggtcacgtgcgtggtggtggacgtgagccaggaagaccccgaggtccagttcaactggtacgtggatggcgtggaggtgcataatgccaagacaaagccgcgggaggagcagttcaacagcacgtaccgtgtggtcagcgtcctcaccgtcctgcaccaggactggctgaacggcaaggagtacaagtgcaaggtctccaacaaaggcctcccgtcctccatcgagaaaaccatctccaaagccaaagggcagccccgagagccacaggtgtacaccctgcccccatcccaggaggagatgaccaagaaccaggtcagcctgacctgcctggtcaaaggcttctaccccagcgacatcgccgtggagtgggagagcaatgggcagccggagaacaactacaagaccacgcctcccgtgctggactccgacggctccttcttcctctacagcaggctcaccgtggacaagagcaggtggcaggaggggaatgtcttctcatgctccgtgatgcatgaggctctgcacaaccactacacacagaagtccctctccctgtctctgggtaaatga

SEQ ID NO: 170 - protein, 452 aa, Homo sapiens
EVQLVESGGRLVQPGGSLRLSCEASGFTFSNYGMTWVRQAPGKGLEWVSVISGSDNRKYYAESVKGRFTISRDNSKNTLYLQMNSLRAEDTAVYYCAKLGYSRSSKDFYYGMDVWGQGTTVTVSSASTKGPSVFPLAPCSRSTSESTAALGCLVKDYFPEPVTVSWNSGALTSGVHTFPAVLQSSGLYSLSSVVTVPSSSLGTKTYTCNVDHKPSNTKVDKRVESKYGPPCPPCPAPEFLGGPSVFLFPPKPKDTLMISRTPEVTCVVVDVSQEDPEVQFNWYVDGVEVHNAKTKPREEQFNSTYRVVSVLTVLHQDWLNGKEYKCKVSNKGLPSSIEKTISKAKGQPREPQVYTLPPSQEEMTKNQVSLTCLVKGFYPSDIAVEWESNGQPENNYKTTPPVLDSDGSFFLYSRLTVDKSRWQEGNVFSCSVMHEALHNHYTQKSLSLSLGK

SEQ ID NO: 171 - DNA, 663 bp, Homo sapiens
gacatcgtgatgacccagtctccagactccctggctgtgtctctgggcgagagggccaccatcaactgcaagtccagccagagtgttttatacaattccaataataggaactacttagtttggtaccagcagaaaccaggacagtctcctaagttgctcatttactgggcatctacccgggaatccggggtccctgaccggttcagtggcagcgggtctgggacagatttcactctcaccatcagcagcctgcaggctgaagatgtggcagtgtattactgtcagcaatattataatgttccgtacacttttggccaggggaccaagctggagatcaaacgaactgtggctgcaccatctgtcttcatcttcccgccatctgatgagcagttgaaatctggaactgcctctgttgtgtgcctgctgaataacttctatcccagagaggccaaagtacagtggaaggtggataacgccctccaatcgggtaactcccaggagagtgtcacagagcaggacagcaaggacagcacctacagcctcagcagcaccctgacgctgagcaaagcagactacgagaaacacaaagtctacgcctgcgaagtcacccatcagggcctgagctcgcccgtcacaaagagcttcaacaggggagagtgttag

SEQ ID NO: 172 - protein, 220 aa, Homo sapiens
DIVMTQSPDSLAVSLGERATINCKSSQSVLYNSNNRNYLVWYQQKPGQSPKLLIYWASTRESGVPDRFSGSGSGTDFTLTISSLQAEDVAVYYCQQYYNVPYTFGQGTKLEIKRTVAAPSVFIFPPSDEQLKSGTASVVCLLNNFYPREAKVQWKVDNALQSGNSQESVTEQDSKDSTYSLSSTLTLSKADYEKHKVYACEVTHQGLSSPVTKSFNRGEC

SEQ ID NO: 173 - DNA, 348 bp, Homo sapiens
gaggtgcagctggtggagtctgggggaggtgtggtacggcctggggggtccctgagactctcctgtgcagcctctggattcacctttgatgattatggcatgagctgggtccgccaagctccagggaaggggctggagtggatctcttctattaataggaatggtggtagcgcagattatgcagactctgtgaagggccgattcaccatctccagagacaacgccaagaactccctctttctgcaaatgagcagtctgagagccgaggacacggccctctatcactgtgcgagcggggagtttcgctttgactactggggccagggaaccctggtcaccgtctcctca

SEQ ID NO: 174 - protein, 116 aa, Homo sapiens
EVQLVESGGGVVRPGGSLRLSCAASGFTFDDYGMSWVRQAPGKGLEWISSINRNGGSADYADSVKGRFTISRDNAKNSLFLQMSSLRAEDTALYHCASGEFRFDYWGQGTLVTVSS

SEQ ID NO: 175 - DNA, 24 bp, Homo sapiens
ggattcacctttgatgattatggc

SEQ ID NO: 176 - protein, 8 aa, Homo sapiens
GFTFDDYG

SEQ ID NO: 177 - DNA, 24 bp, Homo sapiens
attaataggaatggtggtagcgca

SEQ ID NO: 178 - protein, 8 aa, Homo sapiens
INRNGGSA

SEQ ID NO: 179 - DNA, 27 bp, Homo sapiens
gcgagcggggagtttcgctttgactac

SEQ ID NO: 180 - protein, 9 aa, Homo sapiens
ASGEFRFDY

SEQ ID NO: 181 - DNA, 324 bp, Homo sapiens
gacatccagatgacccagtctccatcctccctgtctgcatctgtaggagacagagtcaccatcacttgccgggcaagtcagagcattagcagctatttaaattggtatcagcagaaaccagggaaagcccctaagctcctgatctatgctgcatccagtttgcaaagtggggtcccgtcaaggttcagtggcagtggatctgggacagatttcactctcaccatcagcagtctgcaacctgaagattttgcaacttactactgtcaacagagttacagtacccctccgatcaccttcggccaagggacacgactggagattaaa

SEQ ID NO: 182 - protein, 108 aa, Homo sapiens
DIQMTQSPSSLSASVGDRVTITCRASQSISSYLNWYQQKPGKAPKLLIYAASSLQSGVPSRFSGSGSGTDFTLTISSLQPEDFATYYCQQSYSTPPITFGQGTRLEIK

SEQ ID NO: 183 - DNA, 30 bp, Homo sapiens
caacagagttacagtacccctccgatcacc

SEQ ID NO: 184 - protein, 10 aa, Homo sapiens
QQSYSTPPIT

SEQ ID NO: 185 - DNA, 1332 bp, Homo sapiens
gaggtgcagctggtggagtctgggggaggtgtggtacggcctggggggtccctgagactctcctgtgcagcctctggattcacctttgatgattatggcatgagctgggtccgccaagctccagggaaggggctggagtggatctcttctattaataggaatggtggtagcgcagattatgcagactctgtgaagggccgattcaccatctccagagacaacgccaagaactccctctttctgcaaatgagcagtctgagagccgaggacacggccctctatcactgtgcgagcggggagtttcgctttgactactggggccagggaaccctggtcaccgtctcctcagcctccaccaagggcccatcggtcttccccctggcgccctgctccaggagcacctccgagagcacagccgccctgggctgcctggtcaaggactacttccccgaaccggtgacggtgtcgtggaactcaggcgccctgaccagcggcgtgcacaccttcccggctgtcctacagtcctcaggactctactccctcagcagcgtggtgaccgtgccctccagcagcttgggcacgaagacctacacctgcaacgtagatcacaagcccagcaacaccaaggtggacaagagagttgagtccaaatatggtcccccatgcccaccctgcccagcacctgagttcctggggggaccatcagtcttcctgttccccccaaaacccaaggacactctcatgatctcccggacccctgaggtcacgtgcgtggtggtggacgtgagccaggaagaccccgaggtccagttcaactggtacgtggatggcgtggaggtgcataatgccaagacaaagccgcgggaggagcagttcaacagcacgtaccgtgtggtcagcgtcctcaccgtcctgcaccaggactggctgaacggcaaggagtacaagtgcaaggtctccaacaaaggcctcccgtcctccatcgagaaaaccatctccaaagccaaagggcagccccgagagccacaggtgtacaccctgcccccatcccaggaggagatgaccaagaaccaggtcagcctgacctgcctggtcaaaggcttctaccccagcgacatcgccgtggagtgggagagcaatgggcagccggagaacaactacaagaccacgcctcccgtgctggactccgacggctccttcttcctctacagcaggctcaccgtggacaagagcaggtggcaggaggggaatgtcttctcatgctccgtgatgcatgaggctctgcacaaccactacacacagaagtccctctccctgtctctgggtaaatga

SEQ ID NO: 186 - protein, 443 aa, Homo sapiens
EVQLVESGGGVVRPGGSLRLSCAASGFTFDDYGMSWVRQAPGKGLEWISSINRNGGSADYADSVKGRFTISRDNAKNSLFLQMSSLRAEDTALYHCASGEFRFDYWGQGTLVTVSSASTKGPSVFPLAPCSRSTSESTAALGCLVKDYFPEPVTVSWNSGALTSGVHTFPAVLQSSGLYSLSSVVTVPSSSLGTKTYTCNVDHKPSNTKVDKRVESKYGPPCPPCPAPEFLGGPSVFLFPPKPKDTLMISRTPEVTCVVVDVSQEDPEVQFNWYVDGVEVHNAKTKPREEQFNSTYRVVSVLTVLHQDWLNGKEYKCKVSNKGLPSSIEKTISKAKGQPREPQVYTLPPSQEEMTKNQVSLTCLVKGFYPSDIAVEWESNGQPENNYKTTPPVLDSDGSFFLYSRLTVDKSRWQEGNVFSCSVMHEALHNHYTQKSLSLSLGK

SEQ ID NO: 187 - DNA, 648 bp, Homo sapiens
gacatccagatgacccagtctccatcctccctgtctgcatctgtaggagacagagtcaccatcacttgccgggcaagtcagagcattagcagctatttaaattggtatcagcagaaaccagggaaagcccctaagctcctgatctatgctgcatccagtttgcaaagtggggtcccgtcaaggttcagtggcagtggatctgggacagatttcactctcaccatcagcagtctgcaacctgaagattttgcaacttactactgtcaacagagttacagtacccctccgatcaccttcggccaagggacacgactggagattaaacgaactgtggctgcaccatctgtcttcatcttcccgccatctgatgagcagttgaaatctggaactgcctctgttgtgtgcctgctgaataacttctatcccagagaggccaaagtacagtggaaggtggataacgccctccaatcgggtaactcccaggagagtgtcacagagcaggacagcaaggacagcacctacagcctcagcagcaccctgacgctgagcaaagcagactacgagaaacacaaagtctacgcctgcgaagtcacccatcagggcctgagctcgcccgtcacaaagagcttcaacaggggagagtgttag

SEQ ID NO: 188 - protein, 215 aa, Homo sapiens
DIQMTQSPSSLSASVGDRVTITCRASQSISSYLNWYQQKPGKAPKLLIYAASSLQSGVPSRFSGSGSGTDFTLTISSLQPEDFATYYCQQSYSTPPITFGQGTRLEIKRTVAAPSVFIFPPSDEQLKSGTASVVCLLNNFYPREAKVQWKVDNALQSGNSQESVTEQDSKDSTYSLSSTLTLSKADYEKHKVYACEVTHQGLSSPVTKSFNRGEC

SEQ ID NO: 189 - DNA, 348 bp, Homo sapiens
gaagtgcagctggtggagtctgggggaggcttggtacagcctggcaggtccctgagactctcctgtgcagcctctggattcacccttgaagattatgccatgcactgggtccggcaagctccagggaagggcctggaatgggtctcaggtattagttggaatagaggtagcacaggctatgcggactctgtgaagggccgattcaccatctcaagagacaacgccaagaactccctgtatctgcaaatgaccagtctgagagctgaggacacggccttgtattactgtgcaaaaggattctacagtatggacgtctggggccaagggaccacggtcaccgtctcctca

SEQ ID NO: 190 - protein, 116 aa, Homo sapiens
EVQLVESGGGLVQPGRSLRLSCAASGFTLEDYAMHWVRQAPGKGLEWVSGISWNRGSTGYADSVKGRFTISRDNAKNSLYLQMTSLRAEDTALYYCAKGFYSMDVWGQGTTVTVSS

SEQ ID NO: 191 - DNA, 24 bp, Homo sapiens
ggattcacccttgaagattatgcc

SEQ ID NO: 192 - protein, 8 aa, Homo sapiens
GFTLEDYA

SEQ ID NO: 193 - DNA, 24 bp, Homo sapiens
attagttggaatagaggtagcaca

SEQ ID NO: 194 - protein, 8 aa, Homo sapiens
ISWNRGST

SEQ ID NO: 195 - DNA, 27 bp, Homo sapiens
gcaaaaggattctacagtatggacgtc

SEQ ID NO: 196 - protein, 9 aa, Homo sapiens
AKGFYSMDV

SEQ ID NO: 197 - DNA, 1332 bp, Homo sapiens
gaagtgcagctggtggagtctgggggaggcttggtacagcctggcaggtccctgagactctcctgtgcagcctctggattcacccttgaagattatgccatgcactgggtccggcaagctccagggaagggcctggaatgggtctcaggtattagttggaatagaggtagcacaggctatgcggactctgtgaagggccgattcaccatctcaagagacaacgccaagaactccctgtatctgcaaatgaccagtctgagagctgaggacacggccttgtattactgtgcaaaaggattctacagtatggacgtctggggccaagggaccacggtcaccgtctcctcagcctccaccaagggcccatcggtcttccccctggcgccctgctccaggagcacctccgagagcacagccgccctgggctgcctggtcaaggactacttccccgaaccggtgacggtgtcgtggaactcaggcgccctgaccagcggcgtgcacaccttcccggctgtcctacagtcctcaggactctactccctcagcagcgtggtgaccgtgccctccagcagcttgggcacgaagacctacacctgcaacgtagatcacaagcccagcaacaccaaggtggacaagagagttgagtccaaatatggtcccccatgcccaccctgcccagcacctgagttcctggggggaccatcagtcttcctgttccccccaaaacccaaggacactctcatgatctcccggacccctgaggtcacgtgcgtggtggtggacgtgagccaggaagaccccgaggtccagttcaactggtacgtggatggcgtggaggtgcataatgccaagacaaagccgcgggaggagcagttcaacagcacgtaccgtgtggtcagcgtcctcaccgtcctgcaccaggactggctgaacggcaaggagtacaagtgcaaggtctccaacaaaggcctcccgtcctccatcgagaaaaccatctccaaagccaaagggcagccccgagagccacaggtgtacaccctgcccccatcccaggaggagatgaccaagaaccaggtcagcctgacctgcctggtcaaaggcttctaccccagcgacatcgccgtggagtgggagagcaatgggcagccggagaacaactacaagaccacgcctcccgtgctggactccgacggctccttcttcctctacagcaggctcaccgtggacaagagcaggtggcaggaggggaatgtcttctcatgctccgtgatgcatgaggctctgcacaaccactacacacagaagtccctctccctgtctctgggtaaatga

SEQ ID NO: 198 - protein, 443 aa, Homo sapiens
EVQLVESGGGLVQPGRSLRLSCAASGFTLEDYAMHWVRQAPGKGLEWVSGISWNRGSTGYADSVKGRFTISRDNAKNSLYLQMTSLRAEDTALYYCAKGFYSMDVWGQGTTVTVSSASTKGPSVFPLAPCSRSTSESTAALGCLVKDYFPEPVTVSWNSGALTSGVHTFPAVLQSSGLYSLSSVVTVPSSSLGTKTYTCNVDHKPSNTKVDKRVESKYGPPCPPCPAPEFLGGPSVFLFPPKPKDTLMISRTPEVTCVVVDVSQEDPEVQFNWYVDGVEVHNAKTKPREEQFNSTYRVVSVLTVLHQDWLNGKEYKCKVSNKGLPSSIEKTISKAKGQPREPQVYTLPPSQEEMTKNQVSLTCLVKGFYPSDIAVEWESNGQPENNYKTTPPVLDSDGSFFLYSRLTVDKSRWQEGNVFSCSVMHEALHNHYTQKSLSLSLGK

SEQ ID NO: 199 - DNA, 363 bp, Homo sapiens
caggtacagctgcagcagtcaggtccaggactggtgaagccctcgcagaccctctcactcacctgtgccatctccggtgacagtgtctctagcaacattgctgcttggaactggatcaggctgtccccatcgagaggccttgagtggctgggaaggacattcttcaggtccacgtggttttatgattattcactatctgtgaaaggtcgcataaccatcaacccagacacatccaagaaccagttctccctgcacctgaactctgtgactcccgaggacgcggctgtgtattattgtgcaagaacggggcgacggtggtctcttgactactggggccagggaaccctggtcaccgtctcctca

SEQ ID NO: 200 - protein, 121 aa, Homo sapiens
QVQLQQSGPGLVKPSQTLSLTCAISGDSVSSNIAAWNWIRLSPSRGLEWLGRTFFRSTWFYDYSLSVKGRITINPDTSKNQFSLHLNSVTPEDAAVYYCARTGRRWSLDYWGQGTLVTVSS

SEQ ID NO: 201 - DNA, 30 bp, Homo sapiens
ggtgacagtgtctctagcaacattgctgct

SEQ ID NO: 202 - protein, 10 aa, Homo sapiens
GDSVSSNIAA

SEQ ID NO: 203 - DNA, 27 bp, Homo sapiens
acattcttcaggtccacgtggttttat

SEQ ID NO: 204 - protein, 9 aa, Homo sapiens
TFFRSTWFY

SEQ ID NO: 205 - DNA, 33 bp, Homo sapiens
gcaagaacggggcgacggtggtctcttgactac

SEQ ID NO: 206 - protein, 11 aa, Homo sapiens
ARTGRRWSLDY

SEQ ID NO: 207 - DNA, 1347 bp, Homo sapiens
caggtacagctgcagcagtcaggtccaggactggtgaagccctcgcagaccctctcactcacctgtgccatctccggtgacagtgtctctagcaacattgctgcttggaactggatcaggctgtccccatcgagaggccttgagtggctgggaaggacattcttcaggtccacgtggttttatgattattcactatctgtgaaaggtcgcataaccatcaacccagacacatccaagaaccagttctccctgcacctgaactctgtgactcccgaggacgcggctgtgtattattgtgcaagaacggggcgacggtggtctcttgactactggggccagggaaccctggtcaccgtctcctcagcctccaccaagggcccatcggtcttccccctggcgccctgctccaggagcacctccgagagcacagccgccctgggctgcctggtcaaggactacttccccgaaccggtgacggtgtcgtggaactcaggcgccctgaccagcggcgtgcacaccttcccggctgtcctacagtcctcaggactctactccctcagcagcgtggtgaccgtgccctccagcagcttgggcacgaagacctacacctgcaacgtagatcacaagcccagcaacaccaaggtggacaagagagttgagtccaaatatggtcccccatgcccaccctgcccagcacctgagttcctggggggaccatcagtcttcctgttccccccaaaacccaaggacactctcatgatctcccggacccctgaggtcacgtgcgtggtggtggacgtgagccaggaagaccccgaggtccagttcaactggtacgtggatggcgtggaggtgcataatgccaagacaaagccgcgggaggagcagttcaacagcacgtaccgtgtggtcagcgtcctcaccgtcctgcaccaggactggctgaacggcaaggagtacaagtgcaaggtctccaacaaaggcctcccgtcctccatcgagaaaaccatctccaaagccaaagggcagccccgagagccacaggtgtacaccctgcccccatcccaggaggagatgaccaagaaccaggtcagcctgacctgcctggtcaaaggcttctaccccagcgacatcgccgtggagtgggagagcaatgggcagccggagaacaactacaagaccacgcctcccgtgctggactccgacggctccttcttcctctacagcaggctcaccgtggacaagagcaggtggcaggaggggaatgtcttctcatgctccgtgatgcatgaggctctgcacaaccactacacacagaagtccctctccctgtctctgggtaaatga

SEQ ID NO: 208 - protein, 448 aa, Homo sapiens
QVQLQQSGPGLVKPSQTLSLTCAISGDSVSSNIAAWNWIRLSPSRGLEWLGRTFFRSTWFYDYSLSVKGRITINPDTSKNQFSLHLNSVTPEDAAVYYCARTGRRWSLDYWGQGTLVTVSSASTKGPSVFPLAPCSRSTSESTAALGCLVKDYFPEPVTVSWNSGALTSGVHTFPAVLQSSGLYSLSSVVTVPSSSLGTKTYTCNVDHKPSNTKVDKRVESKYGPPCPPCPAPEFLGGPSVFLFPPKPKDTLMISRTPEVTCVVVDVSQEDPEVQFNWYVDGVEVHNAKTKPREEQFNSTYRVVSVLTVLHQDWLNGKEYKCKVSNKGLPSSIEKTISKAKGQPREPQVYTLPPSQEEMTKNQVSLTCLVKGFYPSDIAVEWESNGQPENNYKTTPPVLDSDGSFFLYSRLTVDKSRWQEGNVFSCSVMHEALHNHYTQKSLSLSLGK

SEQ ID NO: 209 - DNA, 348 bp, Homo sapiens
gaggtgcagctggtggagtctgggggaggtgtggtacggcctggggggtccctgagactctcctgtgcaacctctggattcacctttgatgattatggcatgagctgggtccgccaagttccagggaaggggctggagtgggtctctagtgttaataggaatggtggtaccacagattatgcagactctgtgaagggccgattcaccatctccagagacaatgccaagaggtccctttttctgcaaatgaatagtctgagagccgaagacacggccttgtatcactgtgcgacaggggaacttttctttgactattggggccagggaaccctggtcaccgtctcctca

SEQ ID NO: 210 - protein, 116 aa, Homo sapiens
EVQLVESGGGVVRPGGSLRLSCATSGFTFDDYGMSWVRQVPGKGLEWVSSVNRNGGTTDYADSVKGRFTISRDNAKRSLFLQMNSLRAEDTALYHCATGELFFDYWGQGTLVTVSS

SEQ ID NO: 211 - DNA, 24 bp, Homo sapiens
gttaataggaatggtggtaccaca

SEQ ID NO: 212 - protein, 8 aa, Homo sapiens
VNRNGGTT

SEQ ID NO: 213 - DNA, 27 bp, Homo sapiens
gcgacaggggaacttttctttgactat

SEQ ID NO: 214 - protein, 9 aa, Homo sapiens
ATGELFFDY

SEQ ID NO: 215 - DNA, 1332 bp, Homo sapiens
gaggtgcagctggtggagtctgggggaggtgtggtacggcctggggggtccctgagactctcctgtgcaacctctggattcacctttgatgattatggcatgagctgggtccgccaagttccagggaaggggctggagtgggtctctagtgttaataggaatggtggtaccacagattatgcagactctgtgaagggccgattcaccatctccagagacaatgccaagaggtccctttttctgcaaatgaatagtctgagagccgaagacacggccttgtatcactgtgcgacaggggaacttttctttgactattggggccagggaaccctggtcaccgtctcctcagcctccaccaagggcccatcggtcttccccctggcgccctgctccaggagcacctccgagagcacagccgccctgggctgcctggtcaaggactacttccccgaaccggtgacggtgtcgtggaactcaggcgccctgaccagcggcgtgcacaccttcccggctgtcctacagtcctcaggactctactccctcagcagcgtggtgaccgtgccctccagcagcttgggcacgaagacctacacctgcaacgtagatcacaagcccagcaacaccaaggtggacaagagagttgagtccaaatatggtcccccatgcccaccctgcccagcacctgagttcctggggggaccatcagtcttcctgttccccccaaaacccaaggacactctcatgatctcccggacccctgaggtcacgtgcgtggtggtggacgtgagccaggaagaccccgaggtccagttcaactggtacgtggatggcgtggaggtgcataatgccaagacaaagccgcgggaggagcagttcaacagcacgtaccgtgtggtcagcgtcctcaccgtcctgcaccaggactggctgaacggcaaggagtacaagtgcaaggtctccaacaaaggcctcccgtcctccatcgagaaaaccatctccaaagccaaagggcagccccgagagccacaggtgtacaccctgcccccatcccaggaggagatgaccaagaaccaggtcagcctgacctgcctggtcaaaggcttctaccccagcgacatcgccgtggagtgggagagcaatgggcagccggagaacaactacaagaccacgcctcccgtgctggactccgacggctccttcttcctctacagcaggctcaccgtggacaagagcaggtggcaggaggggaatgtcttctcatgctccgtgatgcatgaggctctgcacaaccactacacacagaagtccctctccctgtctctgggtaaatga

SEQ ID NO: 216 - protein, 443 aa, Homo sapiens
EVQLVESGGGVVRPGGSLRLSCATSGFTFDDYGMSWVRQVPGKGLEWVSSVNRNGGTTDYADSVKGRFTISRDNAKRSLFLQMNSLRAEDTALYHCATGELFFDYWGQGTLVTVSSASTKGPSVFPLAPCSRSTSESTAALGCLVKDYFPEPVTVSWNSGALTSGVHTFPAVLQSSGLYSLSSVVTVPSSSLGTKTYTCNVDHKPSNTKVDKRVESKYGPPCPPCPAPEFLGGPSVFLFPPKPKDTLMISRTPEVTCVVVDVSQEDPEVQFNWYVDGVEVHNAKTKPREEQFNSTYRVVSVLTVLHQDWLNGKEYKCKVSNKGLPSSIEKTISKAKGQPREPQVYTLPPSQEEMTKNQVSLTCLVKGFYPSDIAVEWESNGQPENNYKTTPPVLDSDGSFFLYSRLTVDKSRWQEGNVFSCSVMHEALHNHYTQKSLSLSLGK

SEQ ID NO: 217 - DNA, 357 bp, Homo sapiens
caggtccagctggtacagtctggggctgaggtgaagaagcctggggcctcagtgaaggtctcctgcaaggcttctggatacaccttcaccggccactatatgcactgggtgcgacaggcccctggacaagggcttgagtggatgggatggatctaccctcacagtggtcacacaaattatgcaaagaggtttcagggcagggtcaccatgaccagggacacgtccatcactacagcctacatggagctgatcaggctgagatctgacgacacggccgtgtattactgtgcgagaaggagtgggaggtcctggtatttcgatctgtggggccgtggcaccctggtcactgtctcctca

SEQ ID NO: 218 - protein, 119 aa, Homo sapiens
QVQLVQSGAEVKKPGASVKVSCKASGYTFTGHYMHWVRQAPGQGLEWMGWIYPHSGHTNYAKRFQGRVTMTRDTSITTAYMELIRLRSDDTAVYYCARRSGRSWYFDLWGRGTLVTVSS

SEQ ID NO: 219 - DNA, 24 bp, Homo sapiens
ggatacaccttcaccggccactat

SEQ ID NO: 220 - protein, 8 aa, Homo sapiens
GYTFTGHY

SEQ ID NO: 221 - DNA, 24 bp, Homo sapiens
atctaccctcacagtggtcacaca

SEQ ID NO: 222 - protein, 8 aa, Homo sapiens
IYPHSGHT

SEQ ID NO: 223 - DNA, 36 bp, Homo sapiens
gcgagaaggagtgggaggtcctggtatttcgatctg

SEQ ID NO: 224 - protein, 12 aa, Homo sapiens
ARRSGRSWYFDL

SEQ ID NO: 225 - DNA, 324 bp, Homo sapiens
gaaatagttttgacacagagtcccggcacactgtcactctctcccggggaaagagccaccttgtcatgtagagcaagtcagtcagtctctagctcttatctcgcctggtaccagcagaagccgggacaggcccctagactgctgatctacggggcaagttccagggccaccggaatccccgaccggttcagtggaagcggaagcggaaccgattttactttgacgatttctagactggagccagaggatttcgccgtttactattgtcaacagtacggaagcagcccgtggacgtttggccagggcacgaaggtagaaatcaag

SEQ ID NO: 226 - protein, 108 aa, Homo sapiens
EIVLTQSPGTLSLSPGERATLSCRASQSVSSSYLAWYQQKPGQAPRLLIYGASSRATGIPDRFSGSGSGTDFTLTISRLEPEDFAVYYCQQYGSSPWTFGQGTKVEIK

SEQ ID NO: 227 - DNA, 21 bp, Homo sapiens
cagtcagtctctagctcttat

SEQ ID NO: 228 - protein, 7 aa, Homo sapiens
QSVSSSY

SEQ ID NO: 229 - DNA, 9 bp, Homo sapiens
ggggcaagt

SEQ ID NO: 230 - protein, 3 aa, Homo sapiens
GAS

SEQ ID NO: 231 - DNA, 27 bp, Homo sapiens
caacagtacggaagcagcccgtggacg

SEQ ID NO: 232 - protein, 9 aa, Homo sapiens
QQYGSSPWT

SEQ ID NO: 233 - DNA, 1341 bp, Homo sapiens
caggtccagctggtacagtctggggctgaggtgaagaagcctggggcctcagtgaaggtctcctgcaaggcttctggatacaccttcaccggccactatatgcactgggtgcgacaggcccctggacaagggcttgagtggatgggatggatctaccctcacagtggtcacacaaattatgcaaagaggtttcagggcagggtcaccatgaccagggacacgtccatcactacagcctacatggagctgatcaggctgagatctgacgacacggccgtgtattactgtgcgagaaggagtgggaggtcctggtatttcgatctgtggggccgtggcaccctggtcactgtctcctcagcctccaccaagggcccatcggtcttccccctggcgccctgctccaggagcacctccgagagcacagccgccctgggctgcctggtcaaggactacttccccgaaccggtgacggtgtcgtggaactcaggcgccctgaccagcggcgtgcacaccttcccggctgtcctacagtcctcaggactctactccctcagcagcgtggtgaccgtgccctccagcagcttgggcacgaagacctacacctgcaacgtagatcacaagcccagcaacaccaaggtggacaagagagttgagtccaaatatggtcccccatgcccaccctgcccagcacctgagttcctggggggaccatcagtcttcctgttccccccaaaacccaaggacactctcatgatctcccggacccctgaggtcacgtgcgtggtggtggacgtgagccaggaagaccccgaggtccagttcaactggtacgtggatggcgtggaggtgcataatgccaagacaaagccgcgggaggagcagttcaacagcacgtaccgtgtggtcagcgtcctcaccgtcctgcaccaggactggctgaacggcaaggagtacaagtgcaaggtctccaacaaaggcctcccgtcctccatcgagaaaaccatctccaaagccaaagggcagccccgagagccacaggtgtacaccctgcccccatcccaggaggagatgaccaagaaccaggtcagcctgacctgcctggtcaaaggcttctaccccagcgacatcgccgtggagtgggagagcaatgggcagccggagaacaactacaagaccacgcctcccgtgctggactccgacggctccttcttcctctacagcaggctcaccgtggacaagagcaggtggcaggaggggaatgtcttctcatgctccgtgatgcatgaggctctgcacaaccactacacacagaagtccctctccctgtctctgggtaaatga

SEQ ID NO: 234 - protein, 446 aa, Homo sapiens
QVQLVQSGAEVKKPGASVKVSCKASGYTFTGHYMHWVRQAPGQGLEWMGWIYPHSGHTNYAKRFQGRVTMTRDTSITTAYMELIRLRSDDTAVYYCARRSGRSWYFDLWGRGTLVTVSSASTKGPSVFPLAPCSRSTSESTAALGCLVKDYFPEPVTVSWNSGALTSGVHTFPAVLQSSGLYSLSSVVTVPSSSLGTKTYTCNVDHKPSNTKVDKRVESKYGPPCPPCPAPEFLGGPSVFLFPPKPKDTLMISRTPEVTCVVVDVSQEDPEVQFNWYVDGVEVHNAKTKPREEQFNSTYRVVSVLTVLHQDWLNGKEYKCKVSNKGLPSSIEKTISKAKGQPREPQVYTLPPSQEEMTKNQVSLTCLVKGFYPSDIAVEWESNGQPENNYKTTPPVLDSDGSFFLYSRLTVDKSRWQEGNVFSCSVMHEALHNHYTQKSLSLSLGK

SEQ ID NO: 235 - DNA, 648 bp, Homo sapiens
gaaatagttttgacacagagtcccggcacactgtcactctctcccggggaaagagccaccttgtcatgtagagcaagtcagtcagtctctagctcttatctcgcctggtaccagcagaagccgggacaggcccctagactgctgatctacggggcaagttccagggccaccggaatccccgaccggttcagtggaagcggaagcggaaccgattttactttgacgatttctagactggagccagaggatttcgccgtttactattgtcaacagtacggaagcagcccgtggacgtttggccagggcacgaaggtagaaatcaagcgaactgtggctgcaccatctgtcttcatcttcccgccatctgatgagcagttgaaatctggaactgcctctgttgtgtgcctgctgaataacttctatcccagagaggccaaagtacagtggaaggtggataacgccctccaatcgggtaactcccaggagagtgtcacagagcaggacagcaaggacagcacctacagcctcagcagcaccctgacgctgagcaaagcagactacgagaaacacaaagtctacgcctgcgaagtcacccatcagggcctgagctcgcccgtcacaaagagcttcaacaggggagagtgttag

SEQ ID NO: 236 - protein, 215 aa, Homo sapiens
EIVLTQSPGTLSLSPGERATLSCRASQSVSSSYLAWYQQKPGQAPRLLIYGASSRATGIPDRFSGSGSGTDFTLTISRLEPEDFAVYYCQQYGSSPWTFGQGTKVEIKRTVAAPSVFIFPPSDEQLKSGTASVVCLLNNFYPREAKVQWKVDNALQSGNSQESVTEQDSKDSTYSLSSTLTLSKADYEKHKVYACEVTHQGLSSPVTKSFNRGEC

SEQ ID NO: 237 - DNA, 351 bp, Homo sapiens
gaggtgcagctggtggagtctgggggagggttggtacagcctggggggtccctgggactctcctgtgcagcctctggattcacctttagcaactatgccatgagctgggtccgccaggctccagggaaggggctggagtgggtctcagctgttagtggtggtggtggtggcacatactacgcagactccgtgaagggccggttcaccatctccagagacaattccaagaacacggttcttctgcaaatgaacagcctgagagccgaggacacggccgtatattactgtgcgagaggtcggactgggggccttgactactggggcccgggaaccctggtcaccgtctcctca

SEQ ID NO: 238 - protein, 117 aa, Homo sapiens
EVQLVESGGGLVQPGGSLGLSCAASGFTFSNYAMSWVRQAPGKGLEWVSAVSGGGGGTYYADSVKGRFTISRDNSKNTVLLQMNSLRAEDTAVYYCARGRTGGLDYWGPGTLVTVSS

SEQ ID NO: 239 - DNA, 24 bp, Homo sapiens
ggattcacctttagcaactatgcc

SEQ ID NO: 240 - protein, 8 aa, Homo sapiens
GFTFSNYA

SEQ ID NO: 241 - DNA, 24 bp, Homo sapiens
gttagtggtggtggtggtggcaca

SEQ ID NO: 242 - protein, 8 aa, Homo sapiens
VSGGGGGT

SEQ ID NO: 243 - DNA, 30 bp, Homo sapiens
gcgagaggtcggactgggggccttgactac

SEQ ID NO: 244 - protein, 10 aa, Homo sapiens
ARGRTGGLDY

SEQ ID NO: 245 - DNA, 336 bp, Homo sapiens
gatgttgtgatgactcagtctcctctctccctgcccgtcatctttggacagccggcctccatctcctgcaggtcaagtcaaagcctcgtagacagtgatggaaacacctacttgaattggcttcagcagaggccaggccaatctccaaggcgcctaatttatgaggtttctaaccgggactctggggtcccagacagattcagcggcagtgggtcaggcactgatttcacactgacaatcagcagggtggaggctgaggatgttggcatttattactgcatgcaaggtacgcgctggcctcctactttcggcggagggaccaaggtggagatcaaa

SEQ ID NO: 246 - protein, 112 aa, Homo sapiens
DVVMTQSPLSLPVIFGQPASISCRSSQSLVDSDGNTYLNWLQQRPGQSPRRLIYEVSNRDSGVPDRFSGSGSGTDFTLTISRVEAEDVGIYYCMQGTRWPPTFGGGTKVEIK

SEQ ID NO: 247 - DNA, 33 bp, Homo sapiens
caaagcctcgtagacagtgatggaaacacctac

SEQ ID NO: 248 - protein, 11 aa, Homo sapiens
QSLVDSDGNTY

SEQ ID NO: 249 - DNA, 9 bp, Homo sapiens
gaggtttct

SEQ ID NO: 250 - protein, 3 aa, Homo sapiens
EVS

SEQ ID NO: 251 - DNA, 27 bp, Homo sapiens
atgcaaggtacgcgctggcctcctact

SEQ ID NO: 252 - protein, 9 aa, Homo sapiens
MQGTRWPPT

SEQ ID NO: 253 - DNA, 1335 bp, Homo sapiens
gaggtgcagctggtggagtctgggggagggttggtacagcctggggggtccctgggactctcctgtgcagcctctggattcacctttagcaactatgccatgagctgggtccgccaggctccagggaaggggctggagtgggtctcagctgttagtggtggtggtggtggcacatactacgcagactccgtgaagggccggttcaccatctccagagacaattccaagaacacggttcttctgcaaatgaacagcctgagagccgaggacacggccgtatattactgtgcgagaggtcggactgggggccttgactactggggcccgggaaccctggtcaccgtctcctcagcctccaccaagggcccatcggtcttccccctggcgccctgctccaggagcacctccgagagcacagccgccctgggctgcctggtcaaggactacttccccgaaccggtgacggtgtcgtggaactcaggcgccctgaccagcggcgtgcacaccttcccggctgtcctacagtcctcaggactctactccctcagcagcgtggtgaccgtgccctccagcagcttgggcacgaagacctacacctgcaacgtagatcacaagcccagcaacaccaaggtggacaagagagttgagtccaaatatggtcccccatgcccaccctgcccagcacctgagttcctggggggaccatcagtcttcctgttccccccaaaacccaaggacactctcatgatctcccggacccctgaggtcacgtgcgtggtggtggacgtgagccaggaagaccccgaggtccagttcaactggtacgtggatggcgtggaggtgcataatgccaagacaaagccgcgggaggagcagttcaacagcacgtaccgtgtggtcagcgtcctcaccgtcctgcaccaggactggctgaacggcaaggagtacaagtgcaaggtctccaacaaaggcctcccgtcctccatcgagaaaaccatctccaaagccaaagggcagccccgagagccacaggtgtacaccctgcccccatcccaggaggagatgaccaagaaccaggtcagcctgacctgcctggtcaaaggcttctaccccagcgacatcgccgtggagtgggagagcaatgggcagccggagaacaactacaagaccacgcctcccgtgctggactccgacggctccttcttcctctacagcaggctcaccgtggacaagagcaggtggcaggaggggaatgtcttctcatgctccgtgatgcatgaggctctgcacaaccactacacacagaagtccctctccctgtctctgggtaaatga

SEQ ID NO: 254 - protein, 444 aa, Homo sapiens
EVQLVESGGGLVQPGGSLGLSCAASGFTFSNYAMSWVRQAPGKGLEWVSAVSGGGGGTYYADSVKGRFTISRDNSKNTVLLQMNSLRAEDTAVYYCARGRTGGLDYWGPGTLVTVSSASTKGPSVFPLAPCSRSTSESTAALGCLVKDYFPEPVTVSWNSGALTSGVHTFPAVLQSSGLYSLSSVVTVPSSSLGTKTYTCNVDHKPSNTKVDKRVESKYGPPCPPCPAPEFLGGPSVFLFPPKPKDTLMISRTPEVTCVVVDVSQEDPEVQFNWYVDGVEVHNAKTKPREEQFNSTYRVVSVLTVLHQDWLNGKEYKCKVSNKGLPSSIEKTISKAKGQPREPQVYTLPPSQEEMTKNQVSLTCLVKGFYPSDIAVEWESNGQPENNYKTTPPVLDSDGSFFLYSRLTVDKSRWQEGNVFSCSVMHEALHNHYTQKSLSLSLGK

SEQ ID NO: 255 - DNA, 660 bp, Homo sapiens
gatgttgtgatgactcagtctcctctctccctgcccgtcatctttggacagccggcctccatctcctgcaggtcaagtcaaagcctcgtagacagtgatggaaacacctacttgaattggcttcagcagaggccaggccaatctccaaggcgcctaatttatgaggtttctaaccgggactctggggtcccagacagattcagcggcagtgggtcaggcactgatttcacactgacaatcagcagggtggaggctgaggatgttggcatttattactgcatgcaaggtacgcgctggcctcctactttcggcggagggaccaaggtggagatcaaacgaactgtggctgcaccatctgtcttcatcttcccgccatctgatgagcagttgaaatctggaactgcctctgttgtgtgcctgctgaataacttctatcccagagaggccaaagtacagtggaaggtggataacgccctccaatcgggtaactcccaggagagtgtcacagagcaggacagcaaggacagcacctacagcctcagcagcaccctgacgctgagcaaagcagactacgagaaacacaaagtctacgcctgcgaagtcacccatcagggcctgagctcgcccgtcacaaagagcttcaacaggggagagtgttag

SEQ ID NO: 256 - protein, 219 aa, Homo sapiens
DVVMTQSPLSLPVIFGQPASISCRSSQSLVDSDGNTYLNWLQQRPGQSPRRLIYEVSNRDSGVPDRFSGSGSGTDFTLTISRVEAEDVGIYYCMQGTRWPPTFGGGTKVEIKRTVAAPSVFIFPPSDEQLKSGTASVVCLLNNFYPREAKVQWKVDNALQSGNSQESVTEQDSKDSTYSLSSTLTLSKADYEKHKVYACEVTHQGLSSPVTKSFNRGEC

SEQ ID NO: 257 - DNA, 366 bp, Homo sapiens
gaggtgcagctggtggagtctgggggaggtgtggtccggcctggggggtccctgagactctcctgtgcagcctctggattcatctttgatgattatgacatgagttgggtccgccaacctccagggaggggactggaatgggtctccggtattgattggtttggtggtaccagaggttatgcagactctatgaagggccgattcaccatttccagagacaacgccaagaactccctgtatctgcaaatgaacagcctgagagtcgaggacacggccttctattactgtgcgagagggggggctatagtgggagctgttactccctttgactactggggccagggaaccctggtcactgtctcctca

SEQ ID NO: 258 - protein, 122 aa, Homo sapiens
EVQLVESGGGVVRPGGSLRLSCAASGFIFDDYDMSWVRQPPGRGLEWVSGIDWFGGTRGYADSMKGRFTISRDNAKNSLYLQMNSLRVEDTAFYYCARGGAIVGAVTPFDYWGQGTLVTVSS

SEQ ID NO: 259 - DNA, 24 bp, Homo sapiens
ggattcatctttgatgattatgac

SEQ ID NO: 260 - protein, 8 aa, Homo sapiens
GFIFDDYD

SEQ ID NO: 261 - DNA, 24 bp, Homo sapiens
attgattggtttggtggtaccaga

SEQ ID NO: 262 - protein, 8 aa, Homo sapiens
IDWFGGTR

SEQ ID NO: 263 - DNA, 45 bp, Homo sapiens
gcgagagggggggctatagtgggagctgttactccctttgactac

SEQ ID NO: 264 - protein, 15 aa, Homo sapiens
ARGGAIVGAVTPFDY

SEQ ID NO: 265 - DNA, 321 bp, Homo sapiens
gacatccagatgacccagtctccatcctccctgtctgcatctgttggaaacagagtcaccctcagttgccgggcaagtcagagcattaacacctatttaagttggtatcagcagagaccaggaaaagcccctaagctcctgatctatgctgcatccagtttgcaaagtggggtcccctcaaggttcagtggcagtggagctgggacagatttcactctcaccatcagcagtctgcaacctgaagattttgcaacttactactgtcaacagagttacagtgcccctctcactttcggcggtgggaccaaggtggagatcaaa

SEQ ID NO: 266 - protein, 107 aa, Homo sapiens
DIQMTQSPSSLSASVGNRVTLSCRASQSINTYLSWYQQRPGKAPKLLIYAASSLQSGVPSRFSGSGAGTDFTLTISSLQPEDFATYYCQQSYSAPLTFGGGTKVEIK

SEQ ID NO: 267 - DNA, 18 bp, Homo sapiens
cagagcattaacacctat

SEQ ID NO: 268 - protein, 6 aa, Homo sapiens
QSINTY

SEQ ID NO: 269 - DNA, 27 bp, Homo sapiens
caacagagttacagtgcccctctcact

SEQ ID NO: 270 - protein, 9 aa, Homo sapiens
QQSYSAPLT

SEQ ID NO: 271 - DNA, 1350 bp, Homo sapiens
gaggtgcagctggtggagtctgggggaggtgtggtccggcctggggggtccctgagactctcctgtgcagcctctggattcatctttgatgattatgacatgagttgggtccgccaacctccagggaggggactggaatgggtctccggtattgattggtttggtggtaccagaggttatgcagactctatgaagggccgattcaccatttccagagacaacgccaagaactccctgtatctgcaaatgaacagcctgagagtcgaggacacggccttctattactgtgcgagagggggggctatagtgggagctgttactccctttgactactggggccagggaaccctggtcactgtctcctcagcctccaccaagggcccatcggtcttccccctggcgccctgctccaggagcacctccgagagcacagccgccctgggctgcctggtcaaggactacttccccgaaccggtgacggtgtcgtggaactcaggcgccctgaccagcggcgtgcacaccttcccggctgtcctacagtcctcaggactctactccctcagcagcgtggtgaccgtgccctccagcagcttgggcacgaagacctacacctgcaacgtagatcacaagcccagcaacaccaaggtggacaagagagttgagtccaaatatggtcccccatgcccaccctgcccagcacctgagttcctggggggaccatcagtcttcctgttccccccaaaacccaaggacactctcatgatctcccggacccctgaggtcacgtgcgtggtggtggacgtgagccaggaagaccccgaggtccagttcaactggtacgtggatggcgtggaggtgcataatgccaagacaaagccgcgggaggagcagttcaacagcacgtaccgtgtggtcagcgtcctcaccgtcctgcaccaggactggctgaacggcaaggagtacaagtgcaaggtctccaacaaaggcctcccgtcctccatcgagaaaaccatctccaaagccaaagggcagccccgagagccacaggtgtacaccctgcccccatcccaggaggagatgaccaagaaccaggtcagcctgacctgcctggtcaaaggcttctaccccagcgacatcgccgtggagtgggagagcaatgggcagccggagaacaactacaagaccacgcctcccgtgctggactccgacggctccttcttcctctacagcaggctcaccgtggacaagagcaggtggcaggaggggaatgtcttctcatgctccgtgatgcatgaggctctgcacaaccactacacacagaagtccctctccctgtctctgggtaaatga

SEQ ID NO: 272 - protein, 449 aa, Homo sapiens
EVQLVESGGGVVRPGGSLRLSCAASGFIFDDYDMSWVRQPPGRGLEWVSGIDWFGGTRGYADSMKGRFTISRDNAKNSLYLQMNSLRVEDTAFYYCARGGAIVGAVTPFDYWGQGTLVTVSSASTKGPSVFPLAPCSRSTSESTAALGCLVKDYFPEPVTVSWNSGALTSGVHTFPAVLQSSGLYSLSSVVTVPSSSLGTKTYTCNVDHKPSNTKVDKRVESKYGPPCPPCPAPEFLGGPSVFLFPPKPKDTLMISRTPEVTCVVVDVSQEDPEVQFNWYVDGVEVHNAKTKPREEQFNSTYRVVSVLTVLHQDWLNGKEYKCKVSNKGLPSSIEKTISKAKGQPREPQVYTLPPSQEEMTKNQVSLTCLVKGFYPSDIAVEWESNGQPENNYKTTPPVLDSDGSFFLYSRLTVDKSRWQEGNVFSCSVMHEALHNHYTQKSLSLSLGK

SEQ ID NO: 273 - DNA, 645 bp, Homo sapiens
gacatccagatgacccagtctccatcctccctgtctgcatctgttggaaacagagtcaccctcagttgccgggcaagtcagagcattaacacctatttaagttggtatcagcagagaccaggaaaagcccctaagctcctgatctatgctgcatccagtttgcaaagtggggtcccctcaaggttcagtggcagtggagctgggacagatttcactctcaccatcagcagtctgcaacctgaagattttgcaacttactactgtcaacagagttacagtgcccctctcactttcggcggtgggaccaaggtggagatcaaacgaactgtggctgcaccatctgtcttcatcttcccgccatctgatgagcagttgaaatctggaactgcctctgttgtgtgcctgctgaataacttctatcccagagaggccaaagtacagtggaaggtggataacgccctccaatcgggtaactcccaggagagtgtcacagagcaggacagcaaggacagcacctacagcctcagcagcaccctgacgctgagcaaagcagactacgagaaacacaaagtctacgcctgcgaagtcacccatcagggcctgagctcgcccgtcacaaagagcttcaacaggggagagtgttag

SEQ ID NO: 274 - protein, 214 aa, Homo sapiens
DIQMTQSPSSLSASVGNRVTLSCRASQSINTYLSWYQQRPGKAPKLLIYAASSLQSGVPSRFSGSGAGTDFTLTISSLQPEDFATYYCQQSYSAPLTFGGGTKVEIKRTVAAPSVFIFPPSDEQLKSGTASVVCLLNNFYPREAKVQWKVDNALQSGNSQESVTEQDSKDSTYSLSSTLTLSKADYEKHKVYACEVTHQGLSSPVTKSFNRGEC

SEQ ID NO: 275 - DNA, 366 bp, Homo sapiens
cagctgcagctgcaggagtcgggcccaggactggtgaagccttcggagaccctgtccctcacctgcactgtctctggtggctccatcagcattaagaattactactggggctggatccgtcagcccccagggaaggggctggagtggattgggagtatctattatagtgggaccacctactacaacccgtccctcaagagtcgagtcaccatatccgtagacacgtccaagaaccagttctccctgaagctgagctctgtgaccgccgcagacacggctgtatatcactgtgcgagacatggatacagctatggtcacggctggttcgacccctggggccagggaaccctggtcaccgtctcctca

SEQ ID NO: 276 - protein, 122 aa, Homo sapiens
QLQLQESGPGLVKPSETLSLTCTVSGGSISIKNYYWGWIRQPPGKGLEWIGSIYYSGTTYYNPSLKSRVTISVDTSKNQFSLKLSSVTAADTAVYHCARHGYSYGHGWFDPWGQGTLVTVSS

SEQ ID NO: 277 - DNA, 30 bp, Homo sapiens
ggtggctccatcagcattaagaattactac

SEQ ID NO: 278 - protein, 10 aa, Homo sapiens
GGSISIKNYY

SEQ ID NO: 279 - DNA, 21 bp, Homo sapiens
atctattatagtgggaccacc

SEQ ID NO: 280 - protein, 7 aa, Homo sapiens
IYYSGTT

SEQ ID NO: 281 - DNA, 42 bp, Homo sapiens
gcgagacatggatacagctatggtcacggctggttcgacccc

SEQ ID NO: 282 - protein, 14 aa, Homo sapiens
ARHGYSYGHGWFDP

SEQ ID NO: 283 - DNA, 1350 bp, Homo sapiens
cagctgcagctgcaggagtcgggcccaggactggtgaagccttcggagaccctgtccctcacctgcactgtctctggtggctccatcagcattaagaattactactggggctggatccgtcagcccccagggaaggggctggagtggattgggagtatctattatagtgggaccacctactacaacccgtccctcaagagtcgagtcaccatatccgtagacacgtccaagaaccagttctccctgaagctgagctctgtgaccgccgcagacacggctgtatatcactgtgcgagacatggatacagctatggtcacggctggttcgacccctggggccagggaaccctggtcaccgtctcctcagcctccaccaagggcccatcggtcttccccctggcgccctgctccaggagcacctccgagagcacagccgccctgggctgcctggtcaaggactacttccccgaaccggtgacggtgtcgtggaactcaggcgccctgaccagcggcgtgcacaccttcccggctgtcctacagtcctcaggactctactccctcagcagcgtggtgaccgtgccctccagcagcttgggcacgaagacctacacctgcaacgtagatcacaagcccagcaacaccaaggtggacaagagagttgagtccaaatatggtcccccatgcccaccctgcccagcacctgagttcctggggggaccatcagtcttcctgttccccccaaaacccaaggacactctcatgatctcccggacccctgaggtcacgtgcgtggtggtggacgtgagccaggaagaccccgaggtccagttcaactggtacgtggatggcgtggaggtgcataatgccaagacaaagccgcgggaggagcagttcaacagcacgtaccgtgtggtcagcgtcctcaccgtcctgcaccaggactggctgaacggcaaggagtacaagtgcaaggtctccaacaaaggcctcccgtcctccatcgagaaaaccatctccaaagccaaagggcagccccgagagccacaggtgtacaccctgcccccatcccaggaggagatgaccaagaaccaggtcagcctgacctgcctggtcaaaggcttctaccccagcgacatcgccgtggagtgggagagcaatgggcagccggagaacaactacaagaccacgcctcccgtgctggactccgacggctccttcttcctctacagcaggctcaccgtggacaagagcaggtggcaggaggggaatgtcttctcatgctccgtgatgcatgaggctctgcacaaccactacacacagaagtccctctccctgtctctgggtaaatga

SEQ ID NO: 284 - protein, 449 aa, Homo sapiens
QLQLQESGPGLVKPSETLSLTCTVSGGSISIKNYYWGWIRQPPGKGLEWIGSIYYSGTTYYNPSLKSRVTISVDTSKNQFSLKLSSVTAADTAVYHCARHGYSYGHGWFDPWGQGTLVTVSSASTKGPSVFPLAPCSRSTSESTAALGCLVKDYFPEPVTVSWNSGALTSGVHTFPAVLQSSGLYSLSSVVTVPSSSLGTKTYTCNVDHKPSNTKVDKRVESKYGPPCPPCPAPEFLGGPSVFLFPPKPKDTLMISRTPEVTCVVVDVSQEDPEVQFNWYVDGVEVHNAKTKPREEQFNSTYRVVSVLTVLHQDWLNGKEYKCKVSNKGLPSSIEKTISKAKGQPREPQVYTLPPSQEEMTKNQVSLTCLVKGFYPSDIAVEWESNGQPENNYKTTPPVLDSDGSFFLYSRLTVDKSRWQEGNVFSCSVMHEALHNHYTQKSLSLSLGK

SEQ ID NO: 285 - DNA, 366 bp, Homo sapiens
caggtacagctgcagcagtcaggtccaggactggtaaagccctcacagaccctctcactcacctgtgacatctccggggacagtgtctctagcaacattgctacttggaactggatcaggcagtccccatcgagaggccttgagtggctgggaaggacatattacaggtccaagtggtataaagattatgcagtatctgtgaaaagtcgaataaccatcaacccagacacatccaagaaccagttctccctgcaggtgaactctgtgactcccgaggacacggctgtctattactgtgcaagaatgactgggccgcgatactactttgagtactggggccagggaaccctggtcaccgtctcctca

SEQ ID NO: 286 - protein, 122 aa, Homo sapiens
QVQLQQSGPGLVKPSQTLSLTCDISGDSVSSNIATWNWIRQSPSRGLEWLGRTYYRSKWYKDYAVSVKSRITINPDTSKNQFSLQVNSVTPEDTAVYYCARMTGPRYYFEYWGQGTLVTVSS

SEQ ID NO: 287 - DNA, 30 bp, Homo sapiens
ggggacagtgtctctagcaacattgctact

SEQ ID NO: 288 - protein, 10 aa, Homo sapiens
GDSVSSNIAT

SEQ ID NO: 289 - DNA, 27 bp, Homo sapiens
acatattacaggtccaagtggtataaa

SEQ ID NO: 290 - protein, 9 aa, Homo sapiens
TYYRSKWYK

SEQ ID NO: 291 - DNA, 36 bp, Homo sapiens
gcaagaatgactgggccgcgatactactttgagtac

SEQ ID NO: 292 - protein, 12 aa, Homo sapiens
ARMTGPRYYFEY

SEQ ID NO: 293 - DNA, 1350 bp, Homo sapiens
caggtacagctgcagcagtcaggtccaggactggtaaagccctcacagaccctctcactcacctgtgacatctccggggacagtgtctctagcaacattgctacttggaactggatcaggcagtccccatcgagaggccttgagtggctgggaaggacatattacaggtccaagtggtataaagattatgcagtatctgtgaaaagtcgaataaccatcaacccagacacatccaagaaccagttctccctgcaggtgaactctgtgactcccgaggacacggctgtctattactgtgcaagaatgactgggccgcgatactactttgagtactggggccagggaaccctggtcaccgtctcctcagcctccaccaagggcccatcggtcttccccctggcgccctgctccaggagcacctccgagagcacagccgccctgggctgcctggtcaaggactacttccccgaaccggtgacggtgtcgtggaactcaggcgccctgaccagcggcgtgcacaccttcccggctgtcctacagtcctcaggactctactccctcagcagcgtggtgaccgtgccctccagcagcttgggcacgaagacctacacctgcaacgtagatcacaagcccagcaacaccaaggtggacaagagagttgagtccaaatatggtcccccatgcccaccctgcccagcacctgagttcctggggggaccatcagtcttcctgttccccccaaaacccaaggacactctcatgatctcccggacccctgaggtcacgtgcgtggtggtggacgtgagccaggaagaccccgaggtccagttcaactggtacgtggatggcgtggaggtgcataatgccaagacaaagccgcgggaggagcagttcaacagcacgtaccgtgtggtcagcgtcctcaccgtcctgcaccaggactggctgaacggcaaggagtacaagtgcaaggtctccaacaaaggcctcccgtcctccatcgagaaaaccatctccaaagccaaagggcagccccgagagccacaggtgtacaccctgcccccatcccaggaggagatgaccaagaaccaggtcagcctgacctgcctggtcaaaggcttctaccccagcgacatcgccgtggagtgggagagcaatgggcagccggagaacaactacaagaccacgcctcccgtgctggactccgacggctccttcttcctctacagcaggctcaccgtggacaagagcaggtggcaggaggggaatgtcttctcatgctccgtgatgcatgaggctctgcacaaccactacacacagaagtccctctccctgtctctgggtaaatga

SEQ ID NO: 294 - protein, 449 aa, Homo sapiens
QVQLQQSGPGLVKPSQTLSLTCDISGDSVSSNIATWNWIRQSPSRGLEWLGRTYYRSKWYKDYAVSVKSRITINPDTSKNQFSLQVNSVTPEDTAVYYCARMTGPRYYFEYWGQGTLVTVSSASTKGPSVFPLAPCSRSTSESTAALGCLVKDYFPEPVTVSWNSGALTSGVHTFPAVLQSSGLYSLSSVVTVPSSSLGTKTYTCNVDHKPSNTKVDKRVESKYGPPCPPCPAPEFLGGPSVFLFPPKPKDTLMISRTPEVTCVVVDVSQEDPEVQFNWYVDGVEVHNAKTKPREEQFNSTYRVVSVLTVLHQDWLNGKEYKCKVSNKGLPSSIEKTISKAKGQPREPQVYTLPPSQEEMTKNQVSLTCLVKGFYPSDIAVEWESNGQPENNYKTTPPVLDSDGSFFLYSRLTVDKSRWQEGNVFSCSVMHEALHNHYTQKSLSLSLGK

SEQ ID NO: 295 - DNA, 366 bp, Homo sapiens
gaggtgcagctggtggagtctgggggaggtgtggtccggcctggggggtccctgagactctcctgtgcagcctctggattcacctttgatgattttgacatgagctgggtccgccaaggtccagggaaggggctggagtgggtctctggtattaattggcatgggagtagtacaggttatgcagactctgtgaagggccgattcaccatctccagagacaacgccaagaactccctgtatctgcaaatgagcagtctgagggccgaggacacggccttatatcactgtgtgagaggggggactatagtgggtgccactactccccttgactactggggccagggaaccctggtcaccgtctcctca

SEQ ID NO: 296 - protein, 122 aa, Homo sapiens
EVQLVESGGGVVRPGGSLRLSCAASGFTFDDFDMSWVRQGPGKGLEWVSGINWHGSSTGYADSVKGRFTISRDNAKNSLYLQMSSLRAEDTALYHCVRGGTIVGATTPLDYWGQGTLVTVSS

SEQ ID NO: 297 - DNA, 24 bp, Homo sapiens
ggattcacctttgatgattttgac

SEQ ID NO: 298 - protein, 8 aa, Homo sapiens
GFTFDDFD

SEQ ID NO: 299 - DNA, 24 bp, Homo sapiens
attaattggcatgggagtagtaca

SEQ ID NO: 300 - protein, 8 aa, Homo sapiens
INWHGSST

SEQ ID NO: 301 - DNA, 45 bp, Homo sapiens
gtgagaggggggactatagtgggtgccactactccccttgactac

SEQ ID NO: 302 - protein, 15 aa, Homo sapiens
VRGGTIVGATTPLDY

SEQ ID NO: 303 - DNA, 321 bp, Homo sapiens
gacatccagatgacccagtctccatcctccctgtctgcatctgtaggagacagagtcaccatgacttgccgggcaagtcggaccattagcagctatttaagttggtatcagcagaaatcagggaaagtccctaacctcctgatctttggtgcatccagtttgcaaagtggggtcccatcaaggttcagtgccagtggatctgggacagatttcactctcatcatcagcagtctgcaacctgaagattttgcaacttactactgtcaacagagttacagctcccctctcactttcggcggagggaccaaggtggagatcaaa

SEQ ID NO: 304 - protein, 107 aa, Homo sapiens
DIQMTQSPSSLSASVGDRVTMTCRASRTISSYLSWYQQKSGKVPNLLIFGASSLQSGVPSRFSASGSGTDFTLIISSLQPEDFATYYCQQSYSSPLTFGGGTKVEIK

SEQ ID NO: 305 - DNA, 18 bp, Homo sapiens
cggaccattagcagctat

SEQ ID NO: 306 - protein, 6 aa, Homo sapiens
RTISSY

SEQ ID NO: 307 - DNA, 9 bp, Homo sapiens
ggtgcatcc

SEQ ID NO: 308 - DNA, 27 bp, Homo sapiens
caacagagttacagctcccctctcact

SEQ ID NO: 309 - protein, 9 aa, Homo sapiens
QQSYSSPLT

SEQ ID NO: 310 - DNA, 1350 bp, Homo sapiens
gaggtgcagctggtggagtctgggggaggtgtggtccggcctggggggtccctgagactctcctgtgcagcctctggattcacctttgatgattttgacatgagctgggtccgccaaggtccagggaaggggctggagtgggtctctggtattaattggcatgggagtagtacaggttatgcagactctgtgaagggccgattcaccatctccagagacaacgccaagaactccctgtatctgcaaatgagcagtctgagggccgaggacacggccttatatcactgtgtgagaggggggactatagtgggtgccactactccccttgactactggggccagggaaccctggtcaccgtctcctcagcctccaccaagggcccatcggtcttccccctggcgccctgctccaggagcacctccgagagcacagccgccctgggctgcctggtcaaggactacttccccgaaccggtgacggtgtcgtggaactcaggcgccctgaccagcggcgtgcacaccttcccggctgtcctacagtcctcaggactctactccctcagcagcgtggtgaccgtgccctccagcagcttgggcacgaagacctacacctgcaacgtagatcacaagcccagcaacaccaaggtggacaagagagttgagtccaaatatggtcccccatgcccaccctgcccagcacctgagttcctggggggaccatcagtcttcctgttccccccaaaacccaaggacactctcatgatctcccggacccctgaggtcacgtgcgtggtggtggacgtgagccaggaagaccccgaggtccagttcaactggtacgtggatggcgtggaggtgcataatgccaagacaaagccgcgggaggagcagttcaacagcacgtaccgtgtggtcagcgtcctcaccgtcctgcaccaggactggctgaacggcaaggagtacaagtgcaaggtctccaacaaaggcctcccgtcctccatcgagaaaaccatctccaaagccaaagggcagccccgagagccacaggtgtacaccctgcccccatcccaggaggagatgaccaagaaccaggtcagcctgacctgcctggtcaaaggcttctaccccagcgacatcgccgtggagtgggagagcaatgggcagccggagaacaactacaagaccacgcctcccgtgctggactccgacggctccttcttcctctacagcaggctcaccgtggacaagagcaggtggcaggaggggaatgtcttctcatgctccgtgatgcatgaggctctgcacaaccactacacacagaagtccctctccctgtctctgggtaaatga

SEQ ID NO: 311 - protein, 449 aa, Homo sapiens
EVQLVESGGGVVRPGGSLRLSCAASGFTFDDFDMSWVRQGPGKGLEWVSGINWHGSSTGYADSVKGRFTISRDNAKNSLYLQMSSLRAEDTALYHCVRGGTIVGATTPLDYWGQGTLVTVSSASTKGPSVFPLAPCSRSTSESTAALGCLVKDYFPEPVTVSWNSGALTSGVHTFPAVLQSSGLYSLSSVVTVPSSSLGTKTYTCNVDHKPSNTKVDKRVESKYGPPCPPCPAPEFLGGPSVFLFPPKPKDTLMISRTPEVTCVVVDVSQEDPEVQFNWYVDGVEVHNAKTKPREEQFNSTYRVVSVLTVLHQDWLNGKEYKCKVSNKGLPSSIEKTISKAKGQPREPQVYTLPPSQEEMTKNQVSLTCLVKGFYPSDIAVEWESNGQPENNYKTTPPVLDSDGSFFLYSRLTVDKSRWQEGNVFSCSVMHEALHNHYTQKSLSLSLGK

SEQ ID NO: 312 - DNA, 645 bp, Homo sapiens
gacatccagatgacccagtctccatcctccctgtctgcatctgtaggagacagagtcaccatgacttgccgggcaagtcggaccattagcagctatttaagttggtatcagcagaaatcagggaaagtccctaacctcctgatctttggtgcatccagtttgcaaagtggggtcccatcaaggttcagtgccagtggatctgggacagatttcactctcatcatcagcagtctgcaacctgaagattttgcaacttactactgtcaacagagttacagctcccctctcactttcggcggagggaccaaggtggagatcaaacgaactgtggctgcaccatctgtcttcatcttcccgccatctgatgagcagttgaaatctggaactgcctctgttgtgtgcctgctgaataacttctatcccagagaggccaaagtacagtggaaggtggataacgccctccaatcgggtaactcccaggagagtgtcacagagcaggacagcaaggacagcacctacagcctcagcagcaccctgacgctgagcaaagcagactacgagaaacacaaagtctacgcctgcgaagtcacccatcagggcctgagctcgcccgtcacaaagagcttcaacaggggagagtgttag

SEQ ID NO: 313 - protein, 214 aa, Homo sapiens
DIQMTQSPSSLSASVGDRVTMTCRASRTISSYLSWYQQKSGKVPNLLIFGASSLQSGVPSRFSASGSGTDFTLIISSLQPEDFATYYCQQSYSSPLTFGGGTKVEIKRTVAAPSVFIFPPSDEQLKSGTASVVCLLNNFYPREAKVQWKVDNALQSGNSQESVTEQDSKDSTYSLSSTLTLSKADYEKHKVYACEVTHQGLSSPVTKSFNRGEC

SEQ ID NO: 314 - DNA, 351 bp, Homo sapiens
gaggtgcagctggtggagtctgggggagacttggtacagcctggggggtccctgagactctcctgtacagcctctggattcatttttaggaactatgccatgaactgggtccgccaggctccagggaaggggctggagtggttgtcaggtattcttggtagtaatgataacacatactacgtagactccgtgaagggccggttcaccatttctagagacaattccaggaacacgctgtatctgcaaatgaacagcctgagagccgaggactcggccgtatattactgtgcaaaaggggacgctgggggctttgactactggggccagggaaccctggtcaccgtctcctca

SEQ ID NO: 315 - protein, 117 aa, Homo sapiens
EVQLVESGGDLVQPGGSLRLSCTASGFIFRNYAMNWVRQAPGKGLEWLSGILGSNDNTYYVDSVKGRFTISRDNSRNTLYLQMNSLRAEDSAVYYCAKGDAGGFDYWGQGTLVTVSS

SEQ ID NO: 316 - DNA, 24 bp, Homo sapiens
ggattcatttttaggaactatgcc

SEQ ID NO: 317 - protein, 8 aa, Homo sapiens
GFIFRNYA

SEQ ID NO: 318 - DNA, 24 bp, Homo sapiens
attcttggtagtaatgataacaca

SEQ ID NO: 319 - protein, 8 aa, Homo sapiens
ILGSNDNT

SEQ ID NO: 320 - DNA, 30 bp, Homo sapiens
gcaaaaggggacgctgggggctttgactac

SEQ ID NO: 321 - protein, 10 aa, Homo sapiens
AKGDAGGFDY

SEQ ID NO: 322 - DNA, 336 bp, Homo sapiens
gatgttgtgatgactcagtctccactctccctgcccgtcatccttggacagccggcctccatctcctgcaggtctagtcaaagcctcgtatccagtgatggaaacacctacttgaattggtttcagcagaggccaggccaatctccaaggcgcctaatttataaagtttctaaccgggactctggggtcccagacagattcagcggcagtgggtcaggcactgatttcacactgaaaatcagcagggtggaggctgaggatgttggggcttattactgcatgcaaggttcatactggcctccgacttttggccaggggaccaagctggagatcaaa

SEQ ID NO: 323 - protein, 112 aa, Homo sapiens
DVVMTQSPLSLPVILGQPASISCRSSQSLVSSDGNTYLNWFQQRPGQSPRRLIYKVSNRDSGVPDRFSGSGSGTDFTLKISRVEAEDVGAYYCMQGSYWPPTFGQGTKLEIK

SEQ ID NO: 324 - DNA, 33 bp, Homo sapiens
caaagcctcgtatccagtgatggaaacacctac

SEQ ID NO: 325 - protein, 11 aa, Homo sapiens
QSLVSSDGNTY

SEQ ID NO: 326 - DNA, 9 bp, Homo sapiens
aaagtttct

SEQ ID NO: 327 - protein, 3 aa, Homo sapiens
KVS

SEQ ID NO: 328 - DNA, 27 bp, Homo sapiens
atgcaaggttcatactggcctccgact

SEQ ID NO: 329 - protein, 9 aa, Homo sapiens
MQGSYWPPT

SEQ ID NO: 330 - DNA, 1335 bp, Homo sapiens
gaggtgcagctggtggagtctgggggagacttggtacagcctggggggtccctgagactctcctgtacagcctctggattcatttttaggaactatgccatgaactgggtccgccaggctccagggaaggggctggagtggttgtcaggtattcttggtagtaatgataacacatactacgtagactccgtgaagggccggttcaccatttctagagacaattccaggaacacgctgtatctgcaaatgaacagcctgagagccgaggactcggccgtatattactgtgcaaaaggggacgctgggggctttgactactggggccagggaaccctggtcaccgtctcctcagcctccaccaagggcccatcggtcttccccctggcgccctgctccaggagcacctccgagagcacagccgccctgggctgcctggtcaaggactacttccccgaaccggtgacggtgtcgtggaactcaggcgccctgaccagcggcgtgcacaccttcccggctgtcctacagtcctcaggactctactccctcagcagcgtggtgaccgtgccctccagcagcttgggcacgaagacctacacctgcaacgtagatcacaagcccagcaacaccaaggtggacaagagagttgagtccaaatatggtcccccatgcccaccctgcccagcacctgagttcctggggggaccatcagtcttcctgttccccccaaaacccaaggacactctcatgatctcccggacccctgaggtcacgtgcgtggtggtggacgtgagccaggaagaccccgaggtccagttcaactggtacgtggatggcgtggaggtgcataatgccaagacaaagccgcgggaggagcagttcaacagcacgtaccgtgtggtcagcgtcctcaccgtcctgcaccaggactggctgaacggcaaggagtacaagtgcaaggtctccaacaaaggcctcccgtcctccatcgagaaaaccatctccaaagccaaagggcagccccgagagccacaggtgtacaccctgcccccatcccaggaggagatgaccaagaaccaggtcagcctgacctgcctggtcaaaggcttctaccccagcgacatcgccgtggagtgggagagcaatgggcagccggagaacaactacaagaccacgcctcccgtgctggactccgacggctccttcttcctctacagcaggctcaccgtggacaagagcaggtggcaggaggggaatgtcttctcatgctccgtgatgcatgaggctctgcacaaccactacacacagaagtccctctccctgtctctgggtaaatga

SEQ ID NO: 331 - protein, 444 aa, Homo sapiens
EVQLVESGGDLVQPGGSLRLSCTASGFIFRNYAMNWVRQAPGKGLEWLSGILGSNDNTYYVDSVKGRFTISRDNSRNTLYLQMNSLRAEDSAVYYCAKGDAGGFDYWGQGTLVTVSSASTKGPSVFPLAPCSRSTSESTAALGCLVKDYFPEPVTVSWNSGALTSGVHTFPAVLQSSGLYSLSSVVTVPSSSLGTKTYTCNVDHKPSNTKVDKRVESKYGPPCPPCPAPEFLGGPSVFLFPPKPKDTLMISRTPEVTCVVVDVSQEDPEVQFNWYVDGVEVHNAKTKPREEQFNSTYRVVSVLTVLHQDWLNGKEYKCKVSNKGLPSSIEKTISKAKGQPREPQVYTLPPSQEEMTKNQVSLTCLVKGFYPSDIAVEWESNGQPENNYKTTPPVLDSDGSFFLYSRLTVDKSRWQEGNVFSCSVMHEALHNHYTQKSLSLSLGK

SEQ ID NO: 332 - DNA, 660 bp, Homo sapiens
gatgttgtgatgactcagtctccactctccctgcccgtcatccttggacagccggcctccatctcctgcaggtctagtcaaagcctcgtatccagtgatggaaacacctacttgaattggtttcagcagaggccaggccaatctccaaggcgcctaatttataaagtttctaaccgggactctggggtcccagacagattcagcggcagtgggtcaggcactgatttcacactgaaaatcagcagggtggaggctgaggatgttggggcttattactgcatgcaaggttcatactggcctccgacttttggccaggggaccaagctggagatcaaacgaactgtggctgcaccatctgtcttcatcttcccgccatctgatgagcagttgaaatctggaactgcctctgttgtgtgcctgctgaataacttctatcccagagaggccaaagtacagtggaaggtggataacgccctccaatcgggtaactcccaggagagtgtcacagagcaggacagcaaggacagcacctacagcctcagcagcaccctgacgctgagcaaagcagactacgagaaacacaaagtctacgcctgcgaagtcacccatcagggcctgagctcgcccgtcacaaagagcttcaacaggggagagtgttag

SEQ ID NO: 333 - protein, 219 aa, Homo sapiens
DVVMTQSPLSLPVILGQPASISCRSSQSLVSSDGNTYLNWFQQRPGQSPRRLIYKVSNRDSGVPDRFSGSGSGTDFTLKISRVEAEDVGAYYCMQGSYWPPTFGQGTKLEIKRTVAAPSVFIFPPSDEQLKSGTASVVCLLNNFYPREAKVQWKVDNALQSGNSQESVTEQDSKDSTYSLSSTLTLSKADYEKHKVYACEVTHQGLSSPVTKSFNRGEC

SEQ ID NO: 334 - DNA, 363 bp, Homo sapiens
caggtgcagctggtggagtctgggggaggcgtggtcaagcctggggggtccctgagactctcctgtgcagcctctggattcaccttcagtaactctggcattcactgggtccgccaggctccaggcaaggggctggagtgggtggcacttatatcatatgctggaagtaataaatactatgcagactccgtgaagggccgattcaccatctccagagacaattccaagaacacgctgtctctgcaaatgaacagcctgagagctgaggacacggctgtgtattactgtgcgaaagaggtttggactggaacttatgattcttttgatatgtggggccgagggacaatggtcaccgtctcttca

SEQ ID NO: 335 - protein, 121 aa, Homo sapiens
QVQLVESGGGVVKPGGSLRLSCAASGFTFSNSGIHWVRQAPGKGLEWVALISYAGSNKYYADSVKGRFTISRDNSKNTLSLQMNSLRAEDTAVYYCAKEVWTGTYDSFDMWGRGTMVTVSS

SEQ ID NO: 336 - DNA, 24 bp, Homo sapiens
ggattcaccttcagtaactctggc

SEQ ID NO: 337 - protein, 8 aa, Homo sapiens
GFTFSNSG

SEQ ID NO: 338 - DNA, 24 bp, Homo sapiens
atatcatatgctggaagtaataaa

SEQ ID NO: 339 - protein, 8 aa, Homo sapiens
ISYAGSNK

SEQ ID NO: 340 - DNA, 42 bp, Homo sapiens
gcgaaagaggtttggactggaacttatgattcttttgatatg

SEQ ID NO: 341 - protein, 14 aa, Homo sapiens
AKEVWTGTYDSFDM

SEQ ID NO: 342 - DNA, 1347 bp, Homo sapiens
caggtgcagctggtggagtctgggggaggcgtggtcaagcctggggggtccctgagactctcctgtgcagcctctggattcaccttcagtaactctggcattcactgggtccgccaggctccaggcaaggggctggagtgggtggcacttatatcatatgctggaagtaataaatactatgcagactccgtgaagggccgattcaccatctccagagacaattccaagaacacgctgtctctgcaaatgaacagcctgagagctgaggacacggctgtgtattactgtgcgaaagaggtttggactggaacttatgattcttttgatatgtggggccgagggacaatggtcaccgtctcttcagcctccaccaagggcccatcggtcttccccctggcgccctgctccaggagcacctccgagagcacagccgccctgggctgcctggtcaaggactacttccccgaaccggtgacggtgtcgtggaactcaggcgccctgaccagcggcgtgcacaccttcccggctgtcctacagtcctcaggactctactccctcagcagcgtggtgaccgtgccctccagcagcttgggcacgaagacctacacctgcaacgtagatcacaagcccagcaacaccaaggtggacaagagagttgagtccaaatatggtcccccatgcccaccctgcccagcacctgagttcctggggggaccatcagtcttcctgttccccccaaaacccaaggacactctcatgatctcccggacccctgaggtcacgtgcgtggtggtggacgtgagccaggaagaccccgaggtccagttcaactggtacgtggatggcgtggaggtgcataatgccaagacaaagccgcgggaggagcagttcaacagcacgtaccgtgtggtcagcgtcctcaccgtcctgcaccaggactggctgaacggcaaggagtacaagtgcaaggtctccaacaaaggcctcccgtcctccatcgagaaaaccatctccaaagccaaagggcagccccgagagccacaggtgtacaccctgcccccatcccaggaggagatgaccaagaaccaggtcagcctgacctgcctggtcaaaggcttctaccccagcgacatcgccgtggagtgggagagcaatgggcagccggagaacaactacaagaccacgcctcccgtgctggactccgacggctccttcttcctctacagcaggctcaccgtggacaagagcaggtggcaggaggggaatgtcttctcatgctccgtgatgcatgaggctctgcacaaccactacacacagaagtccctctccctgtctctgggtaaatga

SEQ ID NO: 343 - protein, 448 aa, Homo sapiens
QVQLVESGGGVVKPGGSLRLSCAASGFTFSNSGIHWVRQAPGKGLEWVALISYAGSNKYYADSVKGRFTISRDNSKNTLSLQMNSLRAEDTAVYYCAKEVWTGTYDSFDMWGRGTMVTVSSASTKGPSVFPLAPCSRSTSESTAALGCLVKDYFPEPVTVSWNSGALTSGVHTFPAVLQSSGLYSLSSVVTVPSSSLGTKTYTCNVDHKPSNTKVDKRVESKYGPPCPPCPAPEFLGGPSVFLFPPKPKDTLMISRTPEVTCVVVDVSQEDPEVQFNWYVDGVEVHNAKTKPREEQFNSTYRVVSVLTVLHQDWLNGKEYKCKVSNKGLPSSIEKTISKAKGQPREPQVYTLPPSQEEMTKNQVSLTCLVKGFYPSDIAVEWESNGQPENNYKTTPPVLDSDGSFFLYSRLTVDKSRWQEGNVFSCSVMHEALHNHYTQKSLSLSLGK

SEQ ID NO: 344 - DNA, 363 bp, Homo sapiens
gaggtgcagctggtggagtctgggggaggcttggtacagcctggagggtccctgagactctcctgtgcagcctctggattcatcttcagtagttatgaaatgcattgggtccgccaggctccagggaaggggctggagtggatttcatacattagtagtagtggtactaccatatactacgcagactctgtgaagggccgattcaccatctccagagacaacgccaagaactcactgtatctgcacatgaacagcctgagagccgaggacacggctgtttattactgtacgagagcccgtataactggaactttcgatgtttttgatatctggggccaagggacaatggtcaccgtctcttca

SEQ ID NO: 345 - protein, 121 aa, Homo sapiens
EVQLVESGGGLVQPGGSLRLSCAASGFIFSSYEMHWVRQAPGKGLEWISYISSSGTTIYYADSVKGRFTISRDNAKNSLYLHMNSLRAEDTAVYYCTRARITGTFDVFDIWGQGTMVTVSS

SEQ ID NO: 346 - DNA, 24 bp, Homo sapiens
ggattcatcttcagtagttatgaa

SEQ ID NO: 347 - protein, 8 aa, Homo sapiens
GFIFSSYE

SEQ ID NO: 348 - DNA, 24 bp, Homo sapiens
attagtagtagtggtactaccata

SEQ ID NO: 349 - protein, 8 aa, Homo sapiens
ISSSGTTI

SEQ ID NO: 350 - DNA, 42 bp, Homo sapiens
acgagagcccgtataactggaactttcgatgtttttgatatc

SEQ ID NO: 351 - protein, 14 aa, Homo sapiens
TRARITGTFDVFDI

SEQ ID NO: 352 - DNA, 321 bp, Homo sapiens
gacatccagatgacccagtctccatcctccctgtctgcatctgtgggagacagagtcaccatcacttgccgggcaagtcagagcattagcagctatttaaattggtatcagcagaaaccagggaaagcccctaagctcctgatctttgctgcatccaatttacagagtggggtcccatcaaggttcagtggcagtagatctgggacagatttcactctcaccatcagcagtctgcaacctgaagattttgcaacttactactgtcaacagaattacaatatcccgtacacttttggccaggggaccaagctggagatcaaa

SEQ ID NO: 353 - protein, 107 aa, Homo sapiens
DIQMTQSPSSLSASVGDRVTITCRASQSISSYLNWYQQKPGKAPKLLIFAASNLQSGVPSRFSGSRSGTDFTLTISSLQPEDFATYYCQQNYNIPYTFGQGTKLEIK

SEQ ID NO: 354 - DNA, 27 bp, Homo sapiens
caacagaattacaatatcccgtacact

SEQ ID NO: 355 - protein, 9 aa, Homo sapiens
QQNYNIPYT

SEQ ID NO: 356 - DNA, 1347 bp, Homo sapiens
gaggtgcagctggtggagtctgggggaggcttggtacagcctggagggtccctgagactctcctgtgcagcctctggattcatcttcagtagttatgaaatgcattgggtccgccaggctccagggaaggggctggagtggatttcatacattagtagtagtggtactaccatatactacgcagactctgtgaagggccgattcaccatctccagagacaacgccaagaactcactgtatctgcacatgaacagcctgagagccgaggacacggctgtttattactgtacgagagcccgtataactggaactttcgatgtttttgatatctggggccaagggacaatggtcaccgtctcttcagcctccaccaagggcccatcggtcttccccctggcgccctgctccaggagcacctccgagagcacagccgccctgggctgcctggtcaaggactacttccccgaaccggtgacggtgtcgtggaactcaggcgccctgaccagcggcgtgcacaccttcccggctgtcctacagtcctcaggactctactccctcagcagcgtggtgaccgtgccctccagcagcttgggcacgaagacctacacctgcaacgtagatcacaagcccagcaacaccaaggtggacaagagagttgagtccaaatatggtcccccatgcccaccctgcccagcacctgagttcctggggggaccatcagtcttcctgttccccccaaaacccaaggacactctcatgatctcccggacccctgaggtcacgtgcgtggtggtggacgtgagccaggaagaccccgaggtccagttcaactggtacgtggatggcgtggaggtgcataatgccaagacaaagccgcgggaggagcagttcaacagcacgtaccgtgtggtcagcgtcctcaccgtcctgcaccaggactggctgaacggcaaggagtacaagtgcaaggtctccaacaaaggcctcccgtcctccatcgagaaaaccatctccaaagccaaagggcagccccgagagccacaggtgtacaccctgcccccatcccaggaggagatgaccaagaaccaggtcagcctgacctgcctggtcaaaggcttctaccccagcgacatcgccgtggagtgggagagcaatgggcagccggagaacaactacaagaccacgcctcccgtgctggactccgacggctccttcttcctctacagcaggctcaccgtggacaagagcaggtggcaggaggggaatgtcttctcatgctccgtgatgcatgaggctctgcacaaccactacacacagaagtccctctccctgtctctgggtaaatga

SEQ ID NO: 357 - protein, 448 aa, Homo sapiens
EVQLVESGGGLVQPGGSLRLSCAASGFIFSSYEMHWVRQAPGKGLEWISYISSSGTTIYYADSVKGRFTISRDNAKNSLYLHMNSLRAEDTAVYYCTRARITGTFDVFDIWGQGTMVTVSSASTKGPSVFPLAPCSRSTSESTAALGCLVKDYFPEPVTVSWNSGALTSGVHTFPAVLQSSGLYSLSSVVTVPSSSLGTKTYTCNVDHKPSNTKVDKRVESKYGPPCPPCPAPEFLGGPSVFLFPPKPKDTLMISRTPEVTCVVVDVSQEDPEVQFNWYVDGVEVHNAKTKPREEQFNSTYRVVSVLTVLHQDWLNGKEYKCKVSNKGLPSSIEKTISKAKGQPREPQVYTLPPSQEEMTKNQVSLTCLVKGFYPSDIAVEWESNGQPENNYKTTPPVLDSDGSFFLYSRLTVDKSRWQEGNVFSCSVMHEALHNHYTQKSLSLSLGK

SEQ ID NO: 358 - DNA, 645 bp, Homo sapiens
gacatccagatgacccagtctccatcctccctgtctgcatctgtgggagacagagtcaccatcacttgccgggcaagtcagagcattagcagctatttaaattggtatcagcagaaaccagggaaagcccctaagctcctgatctttgctgcatccaatttacagagtggggtcccatcaaggttcagtggcagtagatctgggacagatttcactctcaccatcagcagtctgcaacctgaagattttgcaacttactactgtcaacagaattacaatatcccgtacacttttggccaggggaccaagctggagatcaaacgaactgtggctgcaccatctgtcttcatcttcccgccatctgatgagcagttgaaatctggaactgcctctgttgtgtgcctgctgaataacttctatcccagagaggccaaagtacagtggaaggtggataacgccctccaatcgggtaactcccaggagagtgtcacagagcaggacagcaaggacagcacctacagcctcagcagcaccctgacgctgagcaaagcagactacgagaaacacaaagtctacgcctgcgaagtcacccatcagggcctgagctcgcccgtcacaaagagcttcaacaggggagagtgttag

SEQ ID NO: 359 - protein, 214 aa, Homo sapiens
DIQMTQSPSSLSASVGDRVTITCRASQSISSYLNWYQQKPGKAPKLLIFAASNLQSGVPSRFSGSRSGTDFTLTISSLQPEDFATYYCQQNYNIPYTFGQGTKLEIKRTVAAPSVFIFPPSDEQLKSGTASVVCLLNNFYPREAKVQWKVDNALQSGNSQESVTEQDSKDSTYSLSSTLTLSKADYEKHKVYACEVTHQGLSSPVTKSFNRGEC

SEQ ID NO: 360 - DNA, 366 bp, Homo sapiens
caggtgcagctgcaggagtcgggcccaggactggtgaagccttcacagaccctgtccctcacctgtactgtctctggtggctccatcaccagtggcggttactactggagctggatccgccagtacccagggcagggcctggagtggattggttacatctattatagtgggaagacctactacaatccgtcttttacgagtcgaattaccatatcagtagacacgtctaagaagcagttctccctgaagatgagctctgtgactgccgcggacacggccgtgtattattgtgcgagagcgggattcacctctagtaacggctggttcgacccctggggccagggaaccctggtcaccgtctcctca

SEQ ID NO: 361 - protein, 122 aa, Homo sapiens
QVQLQESGPGLVKPSQTLSLTCTVSGGSITSGGYYWSWIRQYPGQGLEWIGYIYYSGKTYYNPSFTSRITISVDTSKKQFSLKMSSVTAADTAVYYCARAGFTSSNGWFDPWGQGTLVTVSS

SEQ ID NO: 362 - DNA, 30 bp, Homo sapiens
ggtggctccatcaccagtggcggttactac

SEQ ID NO: 363 - protein, 10 aa, Homo sapiens
GGSITSGGYY

SEQ ID NO: 364 - DNA, 21 bp, Homo sapiens
atctattatagtgggaagacc

SEQ ID NO: 365 - DNA, 42 bp, Homo sapiens
gcgagagcgggattcacctctagtaacggctggttcgacccc

SEQ ID NO: 366 - protein, 14 aa, Homo sapiens
ARAGFTSSNGWFDP

SEQ ID NO: 367 - DNA, 321 bp, Homo sapiens
gacatccagatgacccagtctccatcctccctatctgcatctgtaggagacagagtcaccatcacttgccgggcaagtcagaacattcgcagctatttgaattggtatcagcagaaaccagggaaagccccaaaactcctgatctattctgcatccagtttgcaaagtggggtcccatcaaggttcagtggcagtggatctgggacagatttcactctcaccatcagcagtctgcaacctgaagattttccaacttactactgtcaacagacttacagttccccgtggacgttcggccctgggaccaaggtggaaatcaaa

SEQ ID NO: 368 - protein, 107 aa, Homo sapiens
DIQMTQSPSSLSASVGDRVTITCRASQNIRSYLNWYQQKPGKAPKLLIYSASSLQSGVPSRFSGSGSGTDFTLTISSLQPEDFPTYYCQQTYSSPWTFGPGTKVEIK

SEQ ID NO: 369 - DNA, 18 bp, Homo sapiens
cagaacattcgcagctat

SEQ ID NO: 370 - protein, 6 aa, Homo sapiens
QNIRSY

SEQ ID NO: 371 - DNA, 9 bp, Homo sapiens
tctgcatcc

SEQ ID NO: 372 - protein, 3 aa, Homo sapiens
SAS

SEQ ID NO: 373 - DNA, 27 bp, Homo sapiens
caacagacttacagttccccgtggacg

SEQ ID NO: 374 - protein, 9 aa, Homo sapiens
QQTYSSPWT

SEQ ID NO: 375 - DNA, 1350 bp, Homo sapiens
caggtgcagctgcaggagtcgggcccaggactggtgaagccttcacagaccctgtccctcacctgtactgtctctggtggctccatcaccagtggcggttactactggagctggatccgccagtacccagggcagggcctggagtggattggttacatctattatagtgggaagacctactacaatccgtcttttacgagtcgaattaccatatcagtagacacgtctaagaagcagttctccctgaagatgagctctgtgactgccgcggacacggccgtgtattattgtgcgagagcgggattcacctctagtaacggctggttcgacccctggggccagggaaccctggtcaccgtctcctcagcctccaccaagggcccatcggtcttccccctggcgccctgctccaggagcacctccgagagcacagccgccctgggctgcctggtcaaggactacttccccgaaccggtgacggtgtcgtggaactcaggcgccctgaccagcggcgtgcacaccttcccggctgtcctacagtcctcaggactctactccctcagcagcgtggtgaccgtgccctccagcagcttgggcacgaagacctacacctgcaacgtagatcacaagcccagcaacaccaaggtggacaagagagttgagtccaaatatggtcccccatgcccaccctgcccagcacctgagttcctggggggaccatcagtcttcctgttccccccaaaacccaaggacactctcatgatctcccggacccctgaggtcacgtgcgtggtggtggacgtgagccaggaagaccccgaggtccagttcaactggtacgtggatggcgtggaggtgcataatgccaagacaaagccgcgggaggagcagttcaacagcacgtaccgtgtggtcagcgtcctcaccgtcctgcaccaggactggctgaacggcaaggagtacaagtgcaaggtctccaacaaaggcctcccgtcctccatcgagaaaaccatctccaaagccaaagggcagccccgagagccacaggtgtacaccctgcccccatcccaggaggagatgaccaagaaccaggtcagcctgacctgcctggtcaaaggcttctaccccagcgacatcgccgtggagtgggagagcaatgggcagccggagaacaactacaagaccacgcctcccgtgctggactccgacggctccttcttcctctacagcaggctcaccgtggacaagagcaggtggcaggaggggaatgtcttctcatgctccgtgatgcatgaggctctgcacaaccactacacacagaagtccctctccctgtctctgggtaaatga

SEQ ID NO: 376 - protein, 449 aa, Homo sapiens
QVQLQESGPGLVKPSQTLSLTCTVSGGSITSGGYYWSWIRQYPGQGLEWIGYIYYSGKTYYNPSFTSRITISVDTSKKQFSLKMSSVTAADTAVYYCARAGFTSSNGWFDPWGQGTLVTVSSASTKGPSVFPLAPCSRSTSESTAALGCLVKDYFPEPVTVSWNSGALTSGVHTFPAVLQSSGLYSLSSVVTVPSSSLGTKTYTCNVDHKPSNTKVDKRVESKYGPPCPPCPAPEFLGGPSVFLFPPKPKDTLMISRTPEVTCVVVDVSQEDPEVQFNWYVDGVEVHNAKTKPREEQFNSTYRVVSVLTVLHQDWLNGKEYKCKVSNKGLPSSIEKTISKAKGQPREPQVYTLPPSQEEMTKNQVSLTCLVKGFYPSDIAVEWESNGQPENNYKTTPPVLDSDGSFFLYSRLTVDKSRWQEGNVFSCSVMHEALHNHYTQKSLSLSLGK

SEQ ID NO: 377 - DNA, 645 bp, Homo sapiens
gacatccagatgacccagtctccatcctccctatctgcatctgtaggagacagagtcaccatcacttgccgggcaagtcagaacattcgcagctatttgaattggtatcagcagaaaccagggaaagccccaaaactcctgatctattctgcatccagtttgcaaagtggggtcccatcaaggttcagtggcagtggatctgggacagatttcactctcaccatcagcagtctgcaacctgaagattttccaacttactactgtcaacagacttacagttccccgtggacgttcggccctgggaccaaggtggaaatcaaacgaactgtggctgcaccatctgtcttcatcttcccgccatctgatgagcagttgaaatctggaactgcctctgttgtgtgcctgctgaataacttctatcccagagaggccaaagtacagtggaaggtggataacgccctccaatcgggtaactcccaggagagtgtcacagagcaggacagcaaggacagcacctacagcctcagcagcaccctgacgctgagcaaagcagactacgagaaacacaaagtctacgcctgcgaagtcacccatcagggcctgagctcgcccgtcacaaagagcttcaacaggggagagtgttag

SEQ ID NO: 378 - protein, 214 aa, Homo sapiens
DIQMTQSPSSLSASVGDRVTITCRASQNIRSYLNWYQQKPGKAPKLLIYSASSLQSGVPSRFSGSGSGTDFTLTISSLQPEDFPTYYCQQTYSSPWTFGPGTKVEIKRTVAAPSVFIFPPSDEQLKSGTASVVCLLNNFYPREAKVQWKVDNALQSGNSQESVTEQDSKDSTYSLSSTLTLSKADYEKHKVYACEVTHQGLSSPVTKSFNRGEC

SEQ ID NO: 379 - protein, 268 aa, Artificial Sequence
  Human IL2R extracellular domain expressed with a C-terminal myc-myc-hexahistidine tag
LNTTILTPNGNEDTTADFFLTTMPTDSLSVSTLPLPEVQCFVFNVEYMNCTWNSSSEPQPTNLTLHYWYKNSDNDKVQKCSHYLFSEEITSGCQLQKKEIHLYQTFVVQLQDPREPRRQATQMLKLQNLVIPWAPENLTLHKLSESQLELNWNNRFLNHCLEHLVQYRTDWDHSWTEQSVDYRHKFSLPSVDGQKRYTFRVRSRFNPLCGSAQHWSEWSHPIHWGSNTSKENPFLFALEAEQKLISEEDLGGEQKLISEEDLHHHHHH

SEQ ID NO: 380 - protein, 268 aa, Artificial Sequence
  Macaca fascicularis IL2R extracellular domain expressed with a C-terminal myc-myc-hexahistidine tag
LNTTILTPNGNEDATTDFFLTSMPTDSLSVSTLPLPEVQCFVFNVEYMNCTWNSSSEPQPTNLTLHYWYKNSDNDKVQKCSHYLFSEEITSGCQLQKKEIHLYQTFVVQLQDPREPRRQATQMLKLQNLVIPWAPENLTLRKLSESQLELNWNNRFLNHCLEHLVQYRTDWDHSWTEQSVDYRHKFSLPSVDGQKRYTFRVRSRFNPLCGSAQHWSEWSHPIHWGSNSSKENPFLFALEAEQKLISEEDLGGEQKLISEEDLHHHHHH

SEQ ID NO: 381 - protein, 473 aa, Artificial Sequence
  Human IL2R  extracellular domain expressed with a C-terminal mouse IgG2a Fc tag
LNTTILTPNGNEDTTADFFLTTMPTDSLSVSTLPLPEVQCFVFNVEYMNCTWNSSSEPQPTNLTLHYWYKNSDNDKVQKCSHYLFSEEITSGCQLQKKEIHLYQTFVVQLQDPREPRRQATQMLKLQNLVIPWAPENLTLHKLSESQLELNWNNRFLNHCLEHLVQYRTDWDHSWTEQSVDYRHKFSLPSVDGQKRYTFRVRSRFNPLCGSAQHWSEWSHPIHWGSNTSKENPFLFALEAEPRGPTIKPCPPCKCPAPNLLGGPSVFIFPPKIKDVLMISLSPIVTCVVVDVSEDDPDVQISWFVNNVEVHTAQTQTHREDYNSTLRVVSALPIQHQDWMSGKEFKCKVNNKDLPAPIERTISKPKGSVRAPQVYVLPPPEEEMTKKQVTLTCMVTDFMPEDIYVEWTNNGKTELNYKNTEPVLDSDGSYFMYSKLRVEKKNWVERNSYSCSVVHEGLHNHHTTKSFSRTPGK

SEQ ID NO: 382 - protein, 159 aa, Artificial Sequence
  D1 domain of human IL-2R extracellular domain expressed with a C-terminal myc-myc-hexahistidine tag
LNTTILTPNGNEDTTADFFLTTMPTDSLSVSTLPLPEVQCFVFNVEYMNCTWNSSSEPQPTNLTLHYWYKNSDNDKVQKCSHYLFSEEITSGCQLQKKEIHLYQTFVVQLQDPREPRRQATQMLKLQNLVIEQKLISEEDLGGEQKLISEEDLHHHHHH

SEQ ID NO: 383 - protein, 116 aa, Artificial Sequence
  D2 domain of human IL2R extracellular domain expressed with a C-terminal myc-myc-hexahistidine tag
PWAPENLTLHKLSESQLELNWNNRFLNHCLEHLVQYRTDWDHSWTEQSVDYRHKFSLPSVDGQKRYTFRVRSRFNPLCGSAQHWSEWSEQKLISEEDLGGEQKLISEEDLHHHHHH

SEQ ID NO: 384 - protein, 269 aa, Artificial Sequence
  Mouse IL2R extracellular domain expressed with a C-terminal myc-myc-hexahistidine tag
WSSKVLMSSANEDIKADLILTSTAPEHLSAPTLPLPEVQCFVFNIEYMNCTWNSSSEPQATNLTLHYRYKVSDNNTFQECSHYLFSKEITSGCQIQKEDIQLYQTFVVQLQDPQKPQRRAVQKLNLQNLVIPRAPENLTLSNLSESQLELRWKSRHIKERCLQYLVQYRSNRDRSWTELIVNHEPRFSLPSVDELKRYTFRVRSRYNPICGSSQQWSKWSQPVHWGSHTVEENPSLFALEAEQKLISEEDLGGEQKLISEEDLHHHHHH

SEQ ID NO: 385 - protein, 268 aa, Artificial Sequence
  Rat IL2R extracellular domain expressed with a C-terminal myc-myc-hexahistidine tag
WSSKVLMSSGNEDTKSDLLLTSMDLKHLSVPTLPLPEVQCFVFNVEYMNCTWNSSSEPQPTNLTMHYRYKGSDNNTFQECSHYLFSKEITSGCQIQKEDIQLYQTFVVQLQDPQKPQRRAEQKLNLQNLVIPWAPENLTLYNLSESQVELRWKSRYIERCLQYLVQYRSNRDRSWTEQIVDHEPRFSLPSVDEQKLYTFRVRSRFNPICGSTQQWSKWSQPIHWGSHTAEENPSLFALEAEQKLISEEDLGGEQKLISEEDLHHHHHH

SEQ ID NO: 386 - protein, 5 aa, Artificial Sequence
  G4S linker
GGGGS